European Patent Specification EP 3 618 842 B1, published October 18, 2023. Title: COMBINATION OF A CELL THERAPY AND AN IMMUNOMODULATORY COMPOUND. Applicant: JUNO THERAPEUTICS, INC. PORTS, Michael WORKS, Melissa. Application Not Yet Assigned. The sequence listing filed with the application follows.

SEQUENCE LISTING (189 sequences)

SEQ ID NO: 1 - protein, 12 aa, Homo sapiens
  Spacer (IgG4hinge)
ESKYGPPCPPCP

SEQ ID NO: 2 - DNA, 36 bp, Homo sapiens
  Spacer (IgG4hinge)
gaatctaagtacggaccgccctgccccccttgccct

SEQ ID NO: 3 - protein, 119 aa, Homo sapiens
  Hinge-CH3 spacer
ESKYGPPCPPCPGQPREPQVYTLPPSQEEMTKNQVSLTCLVKGFYPSDIAVEWESNGQPENNYKTTPPVLDSDGSFFLYSRLTVDKSRWQEGNVFSCSVMHEALHNHYTQKSLSLSLGK

SEQ ID NO: 4 - protein, 229 aa, Homo sapiens
  Hinge-CH2-CH3 spacer
ESKYGPPCPPCPAPEFLGGPSVFLFPPKPKDTLMISRTPEVTCVVVDVSQEDPEVQFNWYVDGVEVHNAKTKPREEQFNSTYRVVSVLTVLHQDWLNGKEYKCKVSNKGLPSSIEKTISKAKGQPREPQVYTLPPSQEEMTKNQVSLTCLVKGFYPSDIAVEWESNGQPENNYKTTPPVLDSDGSFFLYSRLTVDKSRWQEGNVFSCSVMHEALHNHYTQKSLSLSLGK

SEQ ID NO: 5 - protein, 282 aa, Homo sapiens
  IgD-hinge-Fc
RWPESPKAQASSVPTAQPQAEGSLAKATTAPATTRNTGRGGEEKKKEKEKEEQEERETKTPECPSHTQPLGVYLLTPAVQDLWLRDKATFTCFVVGSDLKDAHLTWEVAGKVPTGGVEEGLLERHSNGSQSQHSRLTLPRSLWNAGTSVTCTLNHPSLPPQRLMALREPAAQAPVKLSLNLLASSDPPEAASWLLCEVSGFSPPNILLMWLEDQREVNTSGFAPARPPPQPGSTTFWAWSVLRVPAPPSPQPATYTCVVSHEDSRTLLNASRSLEVSYVTDH

SEQ ID NO: 6 - protein, 24 aa, Artificial Sequence
  T2A
LEGGGEGRGSLLTCGDVEENPGPR

SEQ ID NO: 7 - protein, 335 aa, Artificial Sequence
  tEGFR
RKVCNGIGIGEFKDSLSINATNIKHFKNCTSISGDLHILPVAFRGDSFTHTPPLDPQELDILKTVKEITGFLLIQAWPENRTDLHAFENLEIIRGRTKQHGQFSLAVVSLNITSLGLRSLKEISDGDVIISGNKNLCYANTINWKKLFGTSGQKTKIISNRGENSCKATGQVCHALCSPEGCWGPEPRDCVSCRNVSRGRECVDKCNLLEGEPREFVENSECIQCHPECLPQAMNITCTGRGPDNCIQCAHYIDGPHCVKTCPAGVMGENNTLVWKYADAGHVCHLCHPNCTYGCTGPGLEGCPTNGPKIPSIATGMVGALLLLLVVALGIGLFM

SEQ ID NO: 8 - protein, 27 aa, Homo sapiens
  CD28
  ref <308>: UniProt P10747
  ref <309>: 1989-07-01
FWVLVVVGGVLACYSLLVTVAFIIFWV

SEQ ID NO: 9 - protein, 66 aa, Homo sapiens
  CD28
  ref <308>: UniProt P10747
  ref <309>: 1989-07-01
IEVMYPPPYLDNEKSNGTIIHVKGKHLCPSPLFPGPSKPFWVLVVVGGVLACYSLLVTVAFIIFWV

SEQ ID NO: 10 - protein, 41 aa, Homo sapiens
  CD28
  ref <308>: UniProt P10747
  ref <309>: 1989-07-01
RSKRSRLLHSDYMNMTPRRPGPTRKHYQPYAPPRDFAAYRS

SEQ ID NO: 11 - protein, 41 aa, Homo sapiens
  CD28
RSKRSRGGHSDYMNMTPRRPGPTRKHYQPYAPPRDFAAYRS

SEQ ID NO: 12 - protein, 42 aa, Homo sapiens
  4-1BB
  ref <308>: UniProt Q07011.1
  ref <309>: 1995-02-01
KRGRKKLLYIFKQPFMRPVQTTQEEDGCSCRFPEEEEGGCEL

SEQ ID NO: 13 - protein, 112 aa, Homo sapiens
  CD3 zeta
RVKFSRSADAPAYQQGQNQLYNELNLGRREEYDVLDKRRGRDPEMGGKPRRKNPQEGLYNELQKDKMAEAYSEIGMKGERRRGKGHDGLYQGLSTATKDTYDALHMQALPPR

SEQ ID NO: 14 - protein, 112 aa, Homo sapiens
  CD3 zeta
RVKFSRSAEPPAYQQGQNQLYNELNLGRREEYDVLDKRRGRDPEMGGKPRRKNPQEGLYNELQKDKMAEAYSEIGMKGERRRGKGHDGLYQGLSTATKDTYDALHMQALPPR

SEQ ID NO: 15 - protein, 112 aa, Homo sapiens
  CD3 zeta
RVKFSRSADAPAYKQGQNQLYNELNLGRREEYDVLDKRRGRDPEMGGKPRRKNPQEGLYNELQKDKMAEAYSEIGMKGERRRGKGHDGLYQGLSTATKDTYDALHMQALPPR

SEQ ID NO: 16 - protein, 9 aa, Artificial Sequence
  Linker
  REPEAT (5)...(9): SGGGG is repeated 5 times
PGGGSGGGG

SEQ ID NO: 17 - protein, 17 aa, Artificial Sequence
  Linker
GSADDAKKDAAKKDGKS

SEQ ID NO: 18 - protein, 54 aa, Homo sapiens
  Extracellular domain of human BCMA
MLQMAGQCSQNEYFDSLLHACIPCQLRCSSNTPPLTCQRYCNASVTNSVKGTNA

SEQ ID NO: 19 - protein, 5 aa, Artificial Sequence
  Linker
GGGGS

SEQ ID NO: 20 - protein, 231 aa, Artificial Sequence
  Modified Human IgG1 Fc
PKSSDKTHTCPPCPAPEAEGAPSVFLFPPKPKDTLMISRTPEVTCVVVDVSHEDPEVKFNWYVDGVEVHNAKTKPREEQYNSTYRVVSVLTVLHQDWLNGKEYKCKVSNKALPSSIEKTISKAKGQPREPQVYTLPPSRDELTKNQVSLTCLVKGFYPSDIAVEWESNGQPENNYKTTPPVLDSDGSFFLYSKLTVDKSRWQQGNVFSCSVMHEALHNHYTQKSLSLSPGK

SEQ ID NO: 21 - protein, 16 aa, Artificial Sequence
  CD33 Signal peptide
MPLLLLLPLLWAGALA

SEQ ID NO: 22 - protein, 306 aa, Artificial Sequence
  BCMA-Fc
MPLLLLLPLLWAGALAMLQMAGQCSQNEYFDSLLHACIPCQLRCSSNTPPLTCQRYCNASVTNSVKGTNAGGGGSPKSSDKTHTCPPCPAPEAEGAPSVFLFPPKPKDTLMISRTPEVTCVVVDVSHEDPEVKFNWYVDGVEVHNAKTKPREEQYNSTYRVVSVLTVLHQDWLNGKEYKCKVSNKALPSSIEKTISKAKGQPREPQVYTLPPSRDELTKNQVSLTCLVKGFYPSDIAVEWESNGQPENNYKTTPPVLDSDGSFFLYSKLTVDKSRWQQGNVFSCSVMHEALHNHYTQKSLSLSPGK

SEQ ID NO: 23 - protein, 18 aa, Artificial Sequence
  T2A
EGRGSLLTCGDVEENPGP

SEQ ID NO: 24 - protein, 22 aa, Artificial Sequence
  P2A
GSGATNFSLLKQAGDVEENPGP

SEQ ID NO: 25 - protein, 19 aa, Artificial Sequence
  P2A
ATNFSLLKQAGDVEENPGP

SEQ ID NO: 26 - protein, 20 aa, Artificial Sequence
  E2A
QCTNYALLKLAGDVESNPGP

SEQ ID NO: 27 - protein, 22 aa, Artificial Sequence
  F2A
VKQTLNFDLLKLAGDVESNPGP

SEQ ID NO: 28 - protein, 335 aa, Artificial Sequence; identical to SEQ ID NO: 7
  tEGFR

SEQ ID NO: 29 - protein, 228 aa, Homo sapiens
  Hinge-CH2-CH3 spacer
ESKYGPPCPPCPAPPVAGPSVFLFPPKPKDTLMISRTPEVTCVVVDVSQEDPEVQFNWYVDGVEVHNAKTKPREEQFQSTYRVVSVLTVLHQDWLNGKEYKCKVSNKGLPSSIEKTISKAKGQPREPQVYTLPPSQEEMTKNQVSLTCLVKGFYPSDIAVEWESNGQPENNYKTTPPVLDSDGSFFLYSRLTVDKSRWQEGNVFSCSVMHEALHNHYTQKSLSLSLGK

SEQ ID NO: 30 - protein, 117 aa, Artificial Sequence
  Variable heavy (VH) Anti-BCMA
QIQLVQSGPELKKPGETVKISCKASGYTFTDYSINWVKRAPGKGLKWMGWINTETREPAYAYDFRGRFAFSLETSASTAYLQINNLKYEDTATYFCALDYSYAMDYWGQGTSVTVSS

SEQ ID NO: 31 - protein, 111 aa, Artificial Sequence
  Variable light (VL) Anti-BCMA
DIVLTQSPPSLAMSLGKRATISCRASESVTILGSHLIHWYQQKPGQPPTLLIQLASNVQTGVPARFSGSGSRTDFTLTIDPVEEDDVAVYYCLQSRTIPRTFGGGTKLEIK

SEQ ID NO: 32 - protein, 122 aa, Artificial Sequence
  Variable heavy (VH) Anti-BCMA
QIQLVQSGPDLKKPGETVKLSCKASGYTFTNFGMNWVKQAPGKGFKWMAWINTYTGESYFADDFKGRFAFSVETSATTAYLQINNLKTEDTATYFCARGEIYYGYDGGFAYWGQGTLVTVSA

SEQ ID NO: 33 - protein, 107 aa, Artificial Sequence
  Variable light (VL) Anti-BCMA
DVVMTQSHRFMSTSVGDRVSITCRASQDVNTAVSWYQQKPGQSPKLLIFSASYRYTGVPDRFTGSGSGADFTLTISSVQAEDLAVYYCQQHYSTPWTFGGGTKLDIK

SEQ ID NO: 34 - protein, 116 aa, Artificial Sequence
  Variable heavy (VH) Anti-BCMA
EVQLVQSGAEVKKPGESLKISCKGSGYSFTSYWIGWVRQMPGKGLEWMGIIYPGDSDTRYSPSFQGHVTISADKSISTAYLQWSSLKASDTAMYYCARYSGSFDNWGQGTLVTVSS

SEQ ID NO: 35 - protein, 111 aa, Artificial Sequence
  Variable light (VL) Anti-BCMA
SYELTQPPSASGTPGQRVTMSCSGTSSNIGSHSVNWYQQLPGTAPKLLIYTNNQRPSGVPDRFSGSKSGTSASLAISGLQSEDEADYYCAAWDGSLNGLVFGGGTKLTVLG

SEQ ID NO: 36 - protein, 118 aa, Artificial Sequence
  Variable heavy (VH) Anti-BCMA
EVQLVQSGAEMKKPGASLKLSCKASGYTFIDYYVYWMRQAPGQGLESMGWINPNSGGTNYAQKFQGRVTMTRDTSISTAYMELSRLRSDDTAMYYCARSQRDGYMDYWGQGTLVTVSS

SEQ ID NO: 37 - protein, 105 aa, Artificial Sequence
  Variable light (VL) Anti-BCMA
QSALTQPASVSASPGQSIAISCTGTSSDVGWYQQHPGKAPKLMIYEDSKRPSGVSNRFSGSKSGNTASLTISGLQAEDEADYYCSSNTRSSTLVFGGGTKLTVLG

SEQ ID NO: 38 - protein, 122 aa, Artificial Sequence
  Variable heavy (VH) Anti-BCMA
EVQLVQSGAEVKKPGSSVKVSCKASGGTFSSYAISWVRQAPGQGLEWMGRIIPILGIANYAQKFQGRVTMTEDTSTDTAYMELSSLRSEDTAVYYCARSGYSKSIVSYMDYWGQGTLVTVSS

SEQ ID NO: 39 - protein, 111 aa, Artificial Sequence
  Variable light (VL) Anti-BCMA
LPVLTQPPSTSGTPGQRVTVSCSGSSSNIGSNVVFWYQQLPGTAPKLVIYRNNQRPSGVPDRFSVSKSGTSASLAISGLRSEDEADYYCAAWDDSLSGYVFGTGTKVTVLG

SEQ ID NO: 40 - protein, 120 aa, Artificial Sequence
  Variable heavy (VH) Anti-BCMA
QVQLVQSGAEVKKPGSSVKVSCKASGGTFSSYAISWVRQAPGQGLEWMGRIIPILGTANYAQKFQGRVTITADESTSTAYMELSSLRSEDTAVYYCARSGYGSYRWEDSWGQGTLVTVSS

SEQ ID NO: 41 - protein, 112 aa, Artificial Sequence
  Variable light (VL) Anti-BCMA
QAVLTQPPSASGTPGQRVTISCSGSSSNIGSNYVFWYQQLPGTAPKLLIYSNNQRPSGVPDRFSGSKSGTSASLAISGLRSEDEADYYCAAWDDSLSASYVFGTGTKVTVLG

SEQ ID NO: 42 - protein, 118 aa, Artificial Sequence
  Variable heavy (VH) Anti-BCMA
QVQLVQSGAEVKKPGASVKVSCKASGYTFTDYYMHWVRQAPGQRLEWMGWINPNSGGTNYAQKFQDRITVTRDTSSNTGYMELTRLRSDDTAVYYCARSPYSGVLDKWGQGTLVTVSS

SEQ ID NO: 43 - protein, 112 aa, Artificial Sequence
  Variable light (VL) Anti-BCMA
QSVLTQPPSVSGAPGQRVTISCTGSSSNIGAGFDVHWYQQLPGTAPKLLIYGNSNRPSGVPDRFSGSKSGTSASLAITGLQAEDEADYYCQSYDSSLSGYVFGTGTKVTVLG

SEQ ID NO: 44 - protein, 5 aa, Artificial Sequence
  FMC63 CDR H1
DYGVS

SEQ ID NO: 45 - protein, 16 aa, Artificial Sequence
  FMC63 CDR H2
VIWGSETTYYNSALKS

SEQ ID NO: 46 - protein, 7 aa, Artificial Sequence
  FMC63 CDR H3
YAMDYWG

SEQ ID NO: 47 - protein, 12 aa, Artificial Sequence
  FMC63 HC-CDR3
HYYYGGSYAMDY

SEQ ID NO: 48 - protein, 11 aa, Artificial Sequence
  FMC63 CDR L1
RASQDISKYLN

SEQ ID NO: 49 - protein, 7 aa, Artificial Sequence
  FMC63 CDR L2
SRLHSGV

SEQ ID NO: 50 - protein, 7 aa, Artificial Sequence
  FMC63 LC-CDR2
HTSRLHS

SEQ ID NO: 51 - protein, 9 aa, Artificial Sequence
  FMC63 CDR L3
GNTLPYTFG

SEQ ID NO: 52 - protein, 9 aa, Artificial Sequence
  FMC63 LC-CDR3
QQGNTLPYT

SEQ ID NO: 53 - protein, 120 aa, Artificial Sequence
  FMC63 VH
EVKLQESGPGLVAPSQSLSVTCTVSGVSLPDYGVSWIRQPPRKGLEWLGVIWGSETTYYNSALKSRLTIIKDNSKSQVFLKMNSLQTDDTAIYYCAKHYYYGGSYAMDYWGQGTSVTVSS

SEQ ID NO: 54 - protein, 107 aa, Artificial Sequence
  FMC63 VL
DIQMTQTTSSLSASLGDRVTISCRASQDISKYLNWYQQKPDGTVKLLIYHTSRLHSGVPSRFSGSGSGTDYSLTISNLEQEDIATYFCQQGNTLPYTFGGGTKLEIT

SEQ ID NO: 55 - protein, 245 aa, Artificial Sequence
  FMC63 scFv
DIQMTQTTSSLSASLGDRVTISCRASQDISKYLNWYQQKPDGTVKLLIYHTSRLHSGVPSRFSGSGSGTDYSLTISNLEQEDIATYFCQQGNTLPYTFGGGTKLEITGSTSGSGKPGSGEGSTKGEVKLQESGPGLVAPSQSLSVTCTVSGVSLPDYGVSWIRQPPRKGLEWLGVIWGSETTYYNSALKSRLTIIKDNSKSQVFLKMNSLQTDDTAIYYCAKHYYYGGSYAMDYWGQGTSVTVSS

SEQ ID NO: 56 - protein, 11 aa, Artificial Sequence
  SJ25C1 CDR L1
KASQNVGTNVA

SEQ ID NO: 57 - protein, 7 aa, Artificial Sequence
  SJ25C1 CDR L2
SATYRNS

SEQ ID NO: 58 - protein, 9 aa, Artificial Sequence
  SJ25C1 CDR L3
QQYNRYPYT

SEQ ID NO: 59 - protein, 5 aa, Artificial Sequence
  SJ25C1 CDR H1
SYWMN

SEQ ID NO: 60 - protein, 17 aa, Artificial Sequence
  SJ25C1 CDR H2
QIYPGDGDTNYNGKFKG

SEQ ID NO: 61 - protein, 13 aa, Artificial Sequence
  SJ25C1 CDR H3
KTISSVVDFYFDY

SEQ ID NO: 62 - protein, 122 aa, Artificial Sequence
  SJ25C1 VH
EVKLQQSGAELVRPGSSVKISCKASGYAFSSYWMNWVKQRPGQGLEWIGQIYPGDGDTNYNGKFKGQATLTADKSSSTAYMQLSGLTSEDSAVYFCARKTISSVVDFYFDYWGQGTTVTVSS

SEQ ID NO: 63 - protein, 108 aa, Artificial Sequence
  SJ25C1 VL
DIELTQSPKFMSTSVGDRVSVTCKASQNVGTNVAWYQQKPGQSPKPLIYSATYRNSGVPDRFTGSGSGTDFTLTITNVQSKDLADYFCQQYNRYPYTSGGGTKLEIKR

SEQ ID NO: 64 - protein, 15 aa, Artificial Sequence
  Linker
GGGGSGGGGSGGGGS

SEQ ID NO: 65 - protein, 245 aa, Artificial Sequence
  SJ25C1 scFv
EVKLQQSGAELVRPGSSVKISCKASGYAFSSYWMNWVKQRPGQGLEWIGQIYPGDGDTNYNGKFKGQATLTADKSSSTAYMQLSGLTSEDSAVYFCARKTISSVVDFYFDYWGQGTTVTVSSGGGGSGGGGSGGGGSDIELTQSPKFMSTSVGDRVSVTCKASQNVGTNVAWYQQKPGQSPKPLIYSATYRNSGVPDRFTGSGSGTDFTLTITNVQSKDLADYFCQQYNRYPYTSGGGTKLEIKR

SEQ ID NO: 66 - protein, 12 aa, Artificial Sequence
  FMC63 HC-CDR3
HYYYGGSYAMDY

SEQ ID NO: 67 - protein, 7 aa, Artificial Sequence
  FMC63 LC-CDR2
HTSRLHS

SEQ ID NO: 68 - protein, 9 aa, Artificial Sequence
  FMC63 LC-CDR3
QQGNTLPYT

SEQ ID NO: 69 - DNA, 735 bp, Artificial Sequence
  scFv
gacatccagatgacccagaccacctccagcctgagcgccagcctgggcgaccgggtgaccatcagctgccgggccagccaggacatcagcaagtacctgaactggtatcagcagaagcccgacggcaccgtcaagctgctgatctaccacaccagccggctgcacagcggcgtgcccagccggtttagcggcagcggctccggcaccgactacagcctgaccatctccaacctggaacaggaagatatcgccacctacttttgccagcagggcaacacactgccctacacctttggcggcggaacaaagctggaaatcaccggcagcacctccggcagcggcaagcctggcagcggcgagggcagcaccaagggcgaggtgaagctgcaggaaagcggccctggcctggtggcccccagccagagcctgagcgtgacctgcaccgtgagcggcgtgagcctgcccgactacggcgtgagctggatccggcagccccccaggaagggcctggaatggctgggcgtgatctggggcagcgagaccacctactacaacagcgccctgaagagccggctgaccatcatcaaggacaacagcaagagccaggtgttcctgaagatgaacagcctgcagaccgacgacaccgccatctactactgcgccaagcactactactacggcggcagctacgccatggactactggggccagggcaccagcgtgaccgtgagcagc

SEQ ID NO: 70 - protein, 18 aa, Artificial Sequence
  Linker
GSTSGSGKPGSGEGSTKG

SEQ ID NO: 71 - protein, 4 aa, Artificial Sequence
  Linker
GGGS

SEQ ID NO: 72 - protein, 15 aa, Artificial Sequence
  Linker
GGGGSGGGGSGGGGS

SEQ ID NO: 73 - protein, 18 aa, Artificial Sequence
  Linker
GSTSGSGKPGSGEGSTKG

SEQ ID NO: 74 - protein, 21 aa, Artificial Sequence
  Linker
SRGGGGSGGGGSGGGGSLEMA

SEQ ID NO: 75 - protein, 21 aa, Artificial Sequence
  CD8a signal peptide
MALPVTALLLPLALLLHAARP

SEQ ID NO: 76 - protein, 20 aa, Artificial Sequence
  Signal peptide
METDTLLLWVLLLWVPGSTG

SEQ ID NO: 77 - protein, 118 aa, Artificial Sequence
  Variable heavy (VH) Anti-BCMA
EVQLLESGGGLVQPGGSLRLSCAASGFTFSSYAMSWVRQAPGKGLEWVSAISGSGGSTYYADSVKGRFTISRDNSKNTLYLQMNSLRAEDTAVYYCARAEMGAVFDIWGQGTMVTVSS

SEQ ID NO: 78 - protein, 107 aa, Artificial Sequence
  Variable light (VL) Anti-BCMA
EIVLTQSPATLSLSPGERATLSCRASQSVSRYLAWYQQKPGQAPRLLIYDASNRATGIPARFSGSGSGTDFTLTISSLEPEDFAVYYCQQRISWPFTFGGGTKVEIK

SEQ ID NO: 79 - protein, 122 aa, Artificial Sequence
  Variable heavy (VH) Anti-BCMA
QVQLVESGGGVVQPGRSLRLSCAASGFTFSSYGMHWVRQAPGKGLEWVAVISYDGSNKYYADSVKGRFTISRDNSKNTLYLQMNSLRAEDTAVYYCARDGTYLGGLWYFDLWGRGTLVTVSS

SEQ ID NO: 80 - protein, 112 aa, Artificial Sequence
  Variable light (VL) Anti-BCMA
DIVMTQSPLSLPVTPGEPASISCRSSQSLLHSNGYNYLDWYLQKPGQSPQLLIYLGSNRASGVPDRFSGSGSGTDFTLKISRVEAEDVGVYYCMQGLGLPLTFGGGTKVEIK

SEQ ID NO: 81 - protein, 116 aa, Artificial Sequence
  Variable heavy (VH) Anti-BCMA
QVQLVQSGAEVKKPGASVKVSCKASGYTFTSYYMHWVRQAPGQGLEWMGIINPGGGSTSYAQKFQGRVTMTRDTSTSTVYMELSSLRSEDTAVYYCARESWPMDVWGQGTTVTVSS

SEQ ID NO: 82 - protein, 106 aa, Artificial Sequence
  Variable light (VL) Anti-BCMA
EIVMTQSPATLSVSPGERATLSCRASQSVSSNLAWYQQKPGQAPRLLIYGASTRATGIPARFSGSGSGTEFTLTISSLQSEDFAVYYCQQYAAYPTFGGGTKVEIK

SEQ ID NO: 83 - protein, 122 aa, Artificial Sequence
  Variable heavy (VH) Anti-BCMA
QLQLQESGPGLVKPSETLSLTCTVSGGSISSSSYYWGWIRQPPGKGLEWIGSISYSGSTYYNPSLKSRVTISVDTSKNQFSLKLSSVTAADTAVYYCARGRGYATSLAFDIWGQGTMVTVSS

SEQ ID NO: 84 - protein, 107 aa, Artificial Sequence
  Variable light (VL) Anti-BCMA
EIVLTQSPATLSLSPGERATLSCRASQSVSSYLAWYQQKPGQAPRLLIYDASNRATGIPARFSGSGSGTDFTLTISSLEPEDFAVYYCQQRHVWPPTFGGGTKVEIK

SEQ ID NO: 85 - protein, 119 aa, Artificial Sequence
  Variable heavy (VH) Anti-BCMA
EVQLVESGGGLVQPGGSLRLSCAASGFTFSSYSMNWVRQAPGKGLEWVSTISSSSSTIYYADSVKGRFTISRDNAKNSLYLQMNSLRAEDTAVYYCARGSQEHLIFDYWGQGTLVTVSS

SEQ ID NO: 86 - protein, 107 aa, Artificial Sequence
  Variable light (VL) Anti-BCMA
EIVLTQSPATLSLSPGERATLSCRASQSVSRYLAWYQQKPGQAPRLLIYDASNRATGIPARFSGSGSGTDFTLTISSLEPEDFAVYYCQQRFYYPWTFGGGTKVEIK

SEQ ID NO: 87 - protein, 122 aa, Artificial Sequence
  Variable heavy (VH) Anti-BCMA
QVQLVESGGGVVQPGRSLRLSCAASGFTFSSYGMHWVRQAPGKGLEWVAVISYDGSNKYYADSVKGRFTISRDNSKNTLYLQMNSLRAEDTAVYYCARTDFWSGSPPGLDYWGQGTLVTVSS

SEQ ID NO: 88 - protein, 107 aa, Artificial Sequence
  Variable light (VL) Anti-BCMA
DIQLTQSPSSVSASVGDRVTITCRASQGISSWLAWYQQKPGKAPKLLIYGASSLQSGVPSRFSGSGSGTDFTLTISSLQPEDFATYYCQQIYTFPFTFGGGTKVEIK

SEQ ID NO: 89 - protein, 126 aa, Artificial Sequence
  Variable heavy (VH) Anti-BCMA
QVQLVQSGAEVKKPGSSVKVSCKASGGTFSSYAISWVRQAPGQGLEWMGGIIPIFGTANYAQKFQGRVTITADESTSTAYMELSSLRSEDTAVYYCARTPEYSSSIWHYYYGMDVWGQGTTVTVSS

SEQ ID NO: 90 - protein, 113 aa, Artificial Sequence
  Variable light (VL) Anti-BCMA
DIVMTQSPDSLAVSLGERATINCKSSQSVLYSSNNKNYLAWYQQKPGQPPKLLIYWASTRESGVPDRFSGSGSGTDFTLTISSLQAEDVAVYYCQQFAHTPFTFGGGTKVEIK

SEQ ID NO: 91 - protein, 123 aa, Artificial Sequence
  Variable heavy (VH) Anti-BCMA
QVQLVESGGGVVQPGRSLRLSCAASGFTFSSYGMHWVRQAPGKGLEWVAVISYDGSNKYYADSVKGRFTISRDNSKNTLYLQMNSLRAEDTAVYYCVKGPLQEPPYDYGMDVWGQGTTVTVSS

SEQ ID NO: 92 - protein, 107 aa, Artificial Sequence
  Variable light (VL) Anti-BCMA
EIVMTQSPATLSVSPGERATLSCRASQSVSSNLAWYQQKPGQAPRLLIYSASTRATGIPARFSGSGSGTEFTLTISSLQSEDFAVYYCQQHHVWPLTFGGGTKVEIK

SEQ ID NO: 93 - protein, 121 aa, Artificial Sequence
  Variable heavy (VH) Anti-BCMA
QVQLVQSGAEVKKPGSSVKVSCKASGGTFSSYAISWVRQAPGQGLEWMGRIIPILGIANYAQKFQGRVTITADKSTSTAYMELSSLRSEDTAVYYCARGGYYSHDMWSEDWGQGTLVTVSS

SEQ ID NO: 94 - protein, 112 aa, Artificial Sequence
  Variable light (VL) Anti-BCMA
LPVLTQPPSASGTPGQRVTISCSGRSSNIGSNSVNWYRQLPGAAPKLLIYSNNQRPPGVPVRFSGSKSGTSASLAISGLQSEDEATYYCATWDDNLNVHYVFGTGTKVTVLG

SEQ ID NO: 95 - protein, 117 aa, Artificial Sequence
  Variable heavy (VH) Anti-BCMA
QVQLVQSGSELKKPGASVKVSCKASGYTFTDYSINWVRQAPGQGLEWMGWINTETREPAYAYDFRGRFVFSLDTSVSTAYLQISSLKAEDTAVYYCARDYSYAMDYWGQGTLVTVSS

SEQ ID NO: 96 - protein, 111 aa, Artificial Sequence
  Variable light (VL) Anti-BCMA
DIVLTQSPASLAVSLGERATINCRASESVSVIGAHLIHWYQQKPGQPPKLLIYLASNLETGVPARFSGSGSGTDFTLTISSLQAEDAAIYYCLQSRIFPRTFGQGTKLEIK

SEQ ID NO: 97 - protein, 115 aa, Artificial Sequence
  Variable heavy (VH) Anti-BCMA
EVQLVESGGGLVQPGGSLRLSCAVSGFALSNHGMSWVRRAPGKGLEWVSGIVYSGSTYYAASVKGRFTISRDNSRNTLYLQMNSLRPEDTAIYYCSAHGGESDVWGQGTTVTVSS

SEQ ID NO: 98 - protein, 107 aa, Artificial Sequence
  Variable light (VL) Anti-BCMA
DIQLTQSPSSLSASVGDRVTITCRASQSISSYLNWYQQKPGKAPKLLIYAASSLQSGVPSRFSGSGSGTDFTLTISSLQPEDFATYYCQQSYSTPYTFGQGTKVEIK

SEQ ID NO: 99 - protein, 120 aa, Artificial Sequence
  Variable heavy (VH) Anti-BCMA
QVQLVESGGGLVQPGRSLRLSCAASGFTFSNYAMSWVRQAPGKGLGWVSGISRSGENTYYADSVKGRFTISRDNSKNTLYLQMNSLRDEDTAVYYCARSPAHYYGGMDVWGQGTTVTVSS

SEQ ID NO: 100 - protein, 109 aa, Artificial Sequence
  Variable light (VL) Anti-BCMA
DIVLTQSPGTLSLSPGERATLSCRASQSISSSFLAWYQQKPGQAPRLLIYGASRRATGIPDRFSGSGSGTDFTLTISRLEPEDSAVYYCQQYHSSPSWTFGQGTKLEIK

SEQ ID NO: 101 - protein, 115 aa, Artificial Sequence
  Variable heavy (VH) Anti-BCMA
QVQLVESGGGLVQPGGSLRLSCAVSGFALSNHGMSWVRRAPGKGLEWVSGIVYSGSTYYAASVKGRFTISRDNSRNTLYLQMNSLRPEDTAIYYCSAHGGESDVWGQGTTVTVSS

SEQ ID NO: 102 - protein, 107 aa, Artificial Sequence
  Variable light (VL) Anti-BCMA
DIRLTQSPSPLSASVGDRVTITCQASEDINKFLNWYHQTPGKAPKLLIYDASTLQTGVPSRFSGSGSGTDFTLTINSLQPEDIGTYYCQQYESLPLTFGGGTKVEIK

SEQ ID NO: 103 - protein, 115 aa, Artificial Sequence; identical to SEQ ID NO: 97
  Variable heavy (VH) Anti-BCMA

SEQ ID NO: 104 - protein, 109 aa, Artificial Sequence
  Variable light (VL) Anti-BCMA
EIVLTQSPGTLSLSPGERATLSCRASQSIGSSSLAWYQQKPGQAPRLLMYGASSRASGIPDRFSGSGSGTDFTLTISRLEPEDFAVYYCQQYAGSPPFTFGQGTKVEIK

SEQ ID NO: 105 - protein, 117 aa, Artificial Sequence
  Variable heavy (VH) Anti-BCMA
QIQLVQSGPELKKPGETVKISCKASGYTFRHYSMNWVKQAPGKGLKWMGRINTESGVPIYADDFKGRFAFSVETSASTAYLVINNLKDEDTASYFCSNDYLYSLDFWGQGTALTVSS

SEQ ID NO: 106 - protein, 111 aa, Artificial Sequence
  Variable light (VL) Anti-BCMA
DIVLTQSPPSLAMSLGKRATISCRASESVTILGSHLIYWYQQKPGQPPTLLIQLASNVQTGVPARFSGSGSRTDFTLTIDPVEEDDVAVYYCLQSRTIPRTFGGGTKLEIK

SEQ ID NO: 107 - protein, 117 aa, Artificial Sequence
  Variable heavy (VH) Anti-BCMA
QIQLVQSGPELKKPGETVKISCKASGYTFTHYSMNWVKQAPGKGLKWMGRINTETGEPLYADDFKGRFAFSLETSASTAYLVINNLKNEDTATFFCSNDYLYSCDYWGQGTTLTVSS

SEQ ID NO: 108 - protein, 111 aa, Artificial Sequence
  Variable light (VL) Anti-BCMA
DIVLTQSPASLAMSLGKRATISCRASESVSVIGAHLIHWYQQKPGQPPKLLIYLASNLETGVPARFSGSGSGTDFTLTIDPVEEDDVAIYSCLQSRIFPRTFGGGTKLEIK

SEQ ID NO: 109 - protein, 119 aa, Artificial Sequence
  Variable heavy (VH) Anti-BCMA
QVQLVQSGAEVKKPGASVKVSCKASGYSFPDYYINWVRQAPGQGLEWMGWIYFASGNSEYNQKFTGRVTMTRDTSINTAYMELSSLTSEDTAVYFCASLYDYDWYFDVWGQGTMVTVSS

SEQ ID NO: 110 - protein, 112 aa, Artificial Sequence
  Variable light (VL) Anti-BCMA
DIVMTQTPLSLSVTPGQPASISCKSSQSLVHSNGNTYLHWYLQKPGQSPQLLIYKVSNRFSGVPDRFSGSGSGTDFTLKISRVEAEDVGIYYCSQSSIYPWTFGQGTKLEIK

SEQ ID NO: 111 - protein, 119 aa, Artificial Sequence
  Variable heavy (VH) Anti-BCMA
QVQLVQSGAEVKKPGASVKVSCKASGYSFPDYYINWVRQAPGQGLEWMGWIYFASGNSEYNQKFTGRVTMTRDTSSSTAYMELSSLRSEDTAVYFCASLYDYDWYFDVWGQGTMVTVSS

SEQ ID NO: 112 - protein, 112 aa, Artificial Sequence
  Variable light (VL) Anti-BCMA
DIVMTQTPLSLSVTPGEPASISCKSSQSLVHSNGNTYLHWYLQKPGQSPQLLIYKVSNRFSGVPDRFSGSGSGADFTLKISRVEAEDVGVYYCAETSHVPWTFGQGTKLEIK

SEQ ID NO: 113 - protein, 122 aa, Artificial Sequence
  Anti-BCMA sdAb
QVQLVESGGGLVQPGGSLRLSCEASGFTLDYYAIGWFRQAPGKEREGVICISRSDGSTYYADSVKGRFTISRDNAKKTVYLQMISLKPEDTAAYYCAAGADCSGYLRDYEFRGQGTQVTVSS

SEQ ID NO: 114 - protein, 39 aa, Artificial Sequence
  CD28 spacer
IEVMYPPPYLDNEKSNGTIIHVKGKHLCPSPLFPGPSKP

SEQ ID NO: 115 - protein, 25 aa, Artificial Sequence
  CD8a TM
IYIWAPLAGTCGVLLLSLVITLYCN

SEQ ID NO: 116 - protein, 30 aa, Artificial Sequence
  CD28 spacer (truncated)
LDNEKSNGTIIHVKGKHLCPSPLFPGPSKP

SEQ ID NO: 117 - protein, 46 aa, Artificial Sequence
  CD8a hinge
PTTTPAPRPPTPAPTIASQPLSLRPEACRPAAGGAVHTRGLDFACD

SEQ ID NO: 118 - protein, 45 aa, Artificial Sequence
  CD8a hinge
TTTPAPRPPTPAPTIASQPLSLRPEACRPAAGGAVHTRGLDFACD

SEQ ID NO: 119 - protein, 55 aa, Artificial Sequence
  CD8a hinge
FVPVFLPAKPTTTPAPRPPTPAPTIASQPLSLRPEACRPAAGGAVHTRGLDFACD

SEQ ID NO: 120 - protein, 39 aa, Artificial Sequence
  CTLA4 hinge
DTGLYICKVELMYPPPYYLGIGNGTQIYVIDPEPCPDSD

SEQ ID NO: 121 - protein, 24 aa, Artificial Sequence
  CTLA4 TM
FLLWILAAVSSGLFFYSFLLTAVS

SEQ ID NO: 122 - protein, 38 aa, Artificial Sequence
  PD-1 hinge
QIKESLRAELRVTERRAEVPTAHPSPSPRPAGQFQTLV

SEQ ID NO: 123 - protein, 21 aa, Artificial Sequence
  PD-1 TM
VGVVGGLLGSLVLLVWVLAVI

SEQ ID NO: 124 - protein, 16 aa, Artificial Sequence
  Fc(gamma)RIIIa hinge
GLAVSTISSFFPPGYQ

SEQ ID NO: 125 - protein, 231 aa, Artificial Sequence
  IgG1 hinge
EPKSPDKTHTCPPCPAPPVAGPSVFLFPPKPKDTLMIARTPEVTCVVVDVSHEDPEVKFNWYVDGVEVHNAKTKPREEQYNSTYRVVSVLTVLHQDWLNGKEYKCKVSNKALPAPIEKTISKAKGQPREPQVYTLPPSRDELTKNQVSLTCLVKGFYPSDIAVEWESNGQPENNYKTTPPVLDSDGSFFLYSKLTVDKSRWQQGNVFSCSVMHEALHNHYTQKSLSLSPGK

SEQ ID NO: 126 - protein, 457 aa, Artificial Sequence
  anti-BCMA CAR
EVQLLESGGGLVQPGGSLRLSCAASGFTFSSYAMSWVRQAPGKGLEWVSAISGSGGSTYYADSVKGRFTISRDNSKNTLYLQMNSLRAEDTAVYYCARAEMGAVFDIWGQGTMVTVSSGSTSGSGKPGSGEGSTKGEIVLTQSPATLSLSPGERATLSCRASQSVSRYLAWYQQKPGQAPRLLIYDASNRATGIPARFSGSGSGTDFTLTISSLEPEDFAVYYCQQRISWPFTFGGGTKVEIKRAAALDNEKSNGTIIHVKGKHLCPSPLFPGPSKPFWVLVVVGGVLACYSLLVTVAFIIFWVRSKRSRLLHSDYMNMTPRRPGPTRKHYQPYAPPRDFAAYRSRVKFSRSADAPAYQQGQNQLYNELNLGRREEYDVLDKRRGRDPEMGGKPRRKNPQEGLYNELQKDKMAEAYSEIGMKGERRRGKGHDGLYQGLSTATKDTYDALHMQALPPR

SEQ ID NO: 127 - protein, 457 aa, Artificial Sequence
  anti-BCMA CAR
EIVLTQSPATLSLSPGERATLSCRASQSVSRYLAWYQQKPGQAPRLLIYDASNRATGIPARFSGSGSGTDFTLTISSLEPEDFAVYYCQQRISWPFTFGGGTKVEIKRGSTSGSGKPGSGEGSTKGEVQLLESGGGLVQPGGSLRLSCAASGFTFSSYAMSWVRQAPGKGLEWVSAISGSGGSTYYADSVKGRFTISRDNSKNTLYLQMNSLRAEDTAVYYCARAEMGAVFDIWGQGTMVTVSSAAALDNEKSNGTIIHVKGKHLCPSPLFPGPSKPFWVLVVVGGVLACYSLLVTVAFIIFWVRSKRSRLLHSDYMNMTPRRPGPTRKHYQPYAPPRDFAAYRSRVKFSRSADAPAYQQGQNQLYNELNLGRREEYDVLDKRRGRDPEMGGKPRRKNPQEGLYNELQKDKMAEAYSEIGMKGERRRGKGHDGLYQGLSTATKDTYDALHMQALPPR

SEQ ID NO: 128 - protein, 466 aa, Artificial Sequence
  anti-BCMA CAR
QVQLVESGGGVVQPGRSLRLSCAASGFTFSSYGMHWVRQAPGKGLEWVAVISYDGSNKYYADSVKGRFTISRDNSKNTLYLQMNSLRAEDTAVYYCARDGTYLGGLWYFDLWGRGTLVTVSSGSTSGSGKPGSGEGSTKGDIVMTQSPLSLPVTPGEPASISCRSSQSLLHSNGYNYLDWYLQKPGQSPQLLIYLGSNRASGVPDRFSGSGSGTDFTLKISRVEAEDVGVYYCMQGLGLPLTFGGGTKVEIKRAAALDNEKSNGTIIHVKGKHLCPSPLFPGPSKPFWVLVVVGGVLACYSLLVTVAFIIFWVRSKRSRLLHSDYMNMTPRRPGPTRKHYQPYAPPRDFAAYRSRVKFSRSADAPAYQQGQNQLYNELNLGRREEYDVLDKRRGRDPEMGGKPRRKNPQEGLYNELQKDKMAEAYSEIGMKGERRRGKGHDGLYQGLSTATKDTYDALHMQALPPR

SEQ ID NO: 129 - protein, 466 aa, Artificial Sequence
  anti-BCMA CAR
DIVMTQSPLSLPVTPGEPASISCRSSQSLLHSNGYNYLDWYLQKPGQSPQLLIYLGSNRASGVPDRFSGSGSGTDFTLKISRVEAEDVGVYYCMQGLGLPLTFGGGTKVEIKRGSTSGSGKPGSGEGSTKGQVQLVESGGGVVQPGRSLRLSCAASGFTFSSYGMHWVRQAPGKGLEWVAVISYDGSNKYYADSVKGRFTISRDNSKNTLYLQMNSLRAEDTAVYYCARDGTYLGGLWYFDLWGRGTLVTVSSAAALDNEKSNGTIIHVKGKHLCPSPLFPGPSKPFWVLVVVGGVLACYSLLVTVAFIIFWVRSKRSRLLHSDYMNMTPRRPGPTRKHYQPYAPPRDFAAYRSRVKFSRSADAPAYQQGQNQLYNELNLGRREEYDVLDKRRGRDPEMGGKPRRKNPQEGLYNELQKDKMAEAYSEIGMKGERRRGKGHDGLYQGLSTATKDTYDALHMQALPPR

SEQ ID NO: 130 - protein, 454 aa, Artificial Sequence
  anti-BCMA CAR
QVQLVQSGAEVKKPGASVKVSCKASGYTFTSYYMHWVRQAPGQGLEWMGIINPGGGSTSYAQKFQGRVTMTRDTSTSTVYMELSSLRSEDTAVYYCARESWPMDVWGQGTTVTVSSGSTSGSGKPGSGEGSTKGEIVMTQSPATLSVSPGERATLSCRASQSVSSNLAWYQQKPGQAPRLLIYGASTRATGIPARFSGSGSGTEFTLTISSLQSEDFAVYYCQQYAAYPTFGGGTKVEIKRAAALDNEKSNGTIIHVKGKHLCPSPLFPGPSKPFWVLVVVGGVLACYSLLVTVAFIIFWVRSKRSRLLHSDYMNMTPRRPGPTRKHYQPYAPPRDFAAYRSRVKFSRSADAPAYQQGQNQLYNELNLGRREEYDVLDKRRGRDPEMGGKPRRKNPQEGLYNELQKDKMAEAYSEIGMKGERRRGKGHDGLYQGLSTATKDTYDALHMQALPPR

SEQ ID NO: 131 - protein, 454 aa, Artificial Sequence
  anti-BCMA CAR
EIVMTQSPATLSVSPGERATLSCRASQSVSSNLAWYQQKPGQAPRLLIYGASTRATGIPARFSGSGSGTEFTLTISSLQSEDFAVYYCQQYAAYPTFGGGTKVEIKRGSTSGSGKPGSGEGSTKGQVQLVQSGAEVKKPGASVKVSCKASGYTFTSYYMHWVRQAPGQGLEWMGIINPGGGSTSYAQKFQGRVTMTRDTSTSTVYMELSSLRSEDTAVYYCARESWPMDVWGQGTTVTVSSAAALDNEKSNGTIIHVKGKHLCPSPLFPGPSKPFWVLVVVGGVLACYSLLVTVAFIIFWVRSKRSRLLHSDYMNMTPRRPGPTRKHYQPYAPPRDFAAYRSRVKFSRSADAPAYQQGQNQLYNELNLGRREEYDVLDKRRGRDPEMGGKPRRKNPQEGLYNELQKDKMAEAYSEIGMKGERRRGKGHDGLYQGLSTATKDTYDALHMQALPPR

SEQ ID NO: 132 - protein, 461 aa, Artificial Sequence
  anti-BCMA CAR
QLQLQESGPGLVKPSETLSLTCTVSGGSISSSSYYWGWIRQPPGKGLEWIGSISYSGSTYYNPSLKSRVTISVDTSKNQFSLKLSSVTAADTAVYYCARGRGYATSLAFDIWGQGTMVTVSSGSTSGSGKPGSGEGSTKGEIVLTQSPATLSLSPGERATLSCRASQSVSSYLAWYQQKPGQAPRLLIYDASNRATGIPARFSGSGSGTDFTLTISSLEPEDFAVYYCQQRHVWPPTFGGGTKVEIKRAAALDNEKSNGTIIHVKGKHLCPSPLFPGPSKPFWVLVVVGGVLACYSLLVTVAFIIFWVRSKRSRLLHSDYMNMTPRRPGPTRKHYQPYAPPRDFAAYRSRVKFSRSADAPAYQQGQNQLYNELNLGRREEYDVLDKRRGRDPEMGGKPRRKNPQEGLYNELQKDKMAEAYSEIGMKGERRRGKGHDGLYQGLSTATKDTYDALHMQALPPR

SEQ ID NO: 133 - protein, 461 aa, Artificial Sequence
  anti-BCMA CAR
EIVLTQSPATLSLSPGERATLSCRASQSVSSYLAWYQQKPGQAPRLLIYDASNRATGIPARFSGSGSGTDFTLTISSLEPEDFAVYYCQQRHVWPPTFGGGTKVEIKRGSTSGSGKPGSGEGSTKGQLQLQESGPGLVKPSETLSLTCTVSGGSISSSSYYWGWIRQPPGKGLEWIGSISYSGSTYYNPSLKSRVTISVDTSKNQFSLKLSSVTAADTAVYYCARGRGYATSLAFDIWGQGTMVTVSSAAALDNEKSNGTIIHVKGKHLCPSPLFPGPSKPFWVLVVVGGVLACYSLLVTVAFIIFWVRSKRSRLLHSDYMNMTPRRPGPTRKHYQPYAPPRDFAAYRSRVKFSRSADAPAYQQGQNQLYNELNLGRREEYDVLDKRRGRDPEMGGKPRRKNPQEGLYNELQKDKMAEAYSEIGMKGERRRGKGHDGLYQGLSTATKDTYDALHMQALPPR

SEQ ID NO: 134 - protein, 458 aa, Artificial Sequence
  anti-BCMA CAR
EVQLVESGGGLVQPGGSLRLSCAASGFTFSSYSMNWVRQAPGKGLEWVSTISSSSSTIYYADSVKGRFTISRDNAKNSLYLQMNSLRAEDTAVYYCARGSQEHLIFDYWGQGTLVTVSSGSTSGSGKPGSGEGSTKGEIVLTQSPATLSLSPGERATLSCRASQSVSRYLAWYQQKPGQAPRLLIYDASNRATGIPARFSGSGSGTDFTLTISSLEPEDFAVYYCQQRFYYPWTFGGGTKVEIKRAAALDNEKSNGTIIHVKGKHLCPSPLFPGPSKPFWVLVVVGGVLACYSLLVTVAFIIFWVRSKRSRLLHSDYMNMTPRRPGPTRKHYQPYAPPRDFAAYRSRVKFSRSADAPAYQQGQNQLYNELNLGRREEYDVLDKRRGRDPEMGGKPRRKNPQEGLYNELQKDKMAEAYSEIGMKGERRRGKGHDGLYQGLSTATKDTYDALHMQALPPR

SEQ ID NO: 135 - protein, 458 aa, Artificial Sequence
  anti-BCMA CAR
EIVLTQSPATLSLSPGERATLSCRASQSVSRYLAWYQQKPGQAPRLLIYDASNRATGIPARFSGSGSGTDFTLTISSLEPEDFAVYYCQQRFYYPWTFGGGTKVEIKRGSTSGSGKPGSGEGSTKGEVQLVESGGGLVQPGGSLRLSCAASGFTFSSYSMNWVRQAPGKGLEWVSTISSSSSTIYYADSVKGRFTISRDNAKNSLYLQMNSLRAEDTAVYYCARGSQEHLIFDYWGQGTLVTVSSAAALDNEKSNGTIIHVKGKHLCPSPLFPGPSKPFWVLVVVGGVLACYSLLVTVAFIIFWVRSKRSRLLHSDYMNMTPRRPGPTRKHYQPYAPPRDFAAYRSRVKFSRSADAPAYQQGQNQLYNELNLGRREEYDVLDKRRGRDPEMGGKPRRKNPQEGLYNELQKDKMAEAYSEIGMKGERRRGKGHDGLYQGLSTATKDTYDALHMQALPPR

SEQ ID NO: 136 - protein, 461 aa, Artificial Sequence
  anti-BCMA CAR
QVQLVESGGGVVQPGRSLRLSCAASGFTFSSYGMHWVRQAPGKGLEWVAVISYDGSNKYYADSVKGRFTISRDNSKNTLYLQMNSLRAEDTAVYYCARTDFWSGSPPGLDYWGQGTLVTVSSGSTSGSGKPGSGEGSTKGDIQLTQSPSSVSASVGDRVTITCRASQGISSWLAWYQQKPGKAPKLLIYGASSLQSGVPSRFSGSGSGTDFTLTISSLQPEDFATYYCQQIYTFPFTFGGGTKVEIKRAAALDNEKSNGTIIHVKGKHLCPSPLFPGPSKPFWVLVVVGGVLACYSLLVTVAFIIFWVRSKRSRLLHSDYMNMTPRRPGPTRKHYQPYAPPRDFAAYRSRVKFSRSADAPAYQQGQNQLYNELNLGRREEYDVLDKRRGRDPEMGGKPRRKNPQEGLYNELQKDKMAEAYSEIGMKGERRRGKGHDGLYQGLSTATKDTYDALHMQALPPR

SEQ ID NO: 137 - protein, 461 aa, Artificial Sequence
  anti-BCMA CAR
DIQLTQSPSSVSASVGDRVTITCRASQGISSWLAWYQQKPGKAPKLLIYGASSLQSGVPSRFSGSGSGTDFTLTISSLQPEDFATYYCQQIYTFPFTFGGGTKVEIKRGSTSGSGKPGSGEGSTKGQVQLVESGGGVVQPGRSLRLSCAASGFTFSSYGMHWVRQAPGKGLEWVAVISYDGSNKYYADSVKGRFTISRDNSKNTLYLQMNSLRAEDTAVYYCARTDFWSGSPPGLDYWGQGTLVTVSSAAALDNEKSNGTIIHVKGKHLCPSPLFPGPSKPFWVLVVVGGVLACYSLLVTVAFIIFWVRSKRSRLLHSDYMNMTPRRPGPTRKHYQPYAPPRDFAAYRSRVKFSRSADAPAYQQGQNQLYNELNLGRREEYDVLDKRRGRDPEMGGKPRRKNPQEGLYNELQKDKMAEAYSEIGMKGERRRGKGHDGLYQGLSTATKDTYDALHMQALPPR

SEQ ID NO: 138 - protein, 471 aa, Artificial Sequence
  anti-BCMA CAR
QVQLVQSGAEVKKPGSSVKVSCKASGGTFSSYAISWVRQAPGQGLEWMGGIIPIFGTANYAQKFQGRVTITADESTSTAYMELSSLRSEDTAVYYCARTPEYSSSIWHYYYGMDVWGQGTTVTVSSGSTSGSGKPGSGEGSTKGDIVMTQSPDSLAVSLGERATINCKSSQSVLYSSNNKNYLAWYQQKPGQPPKLLIYWASTRESGVPDRFSGSGSGTDFTLTISSLQAEDVAVYYCQQFAHTPFTFGGGTKVEIKRAAALDNEKSNGTIIHVKGKHLCPSPLFPGPSKPFWVLVVVGGVLACYSLLVTVAFIIFWVRSKRSRLLHSDYMNMTPRRPGPTRKHYQPYAPPRDFAAYRSRVKFSRSADAPAYQQGQNQLYNELNLGRREEYDVLDKRRGRDPEMGGKPRRKNPQEGLYNELQKDKMAEAYSEIGMKGERRRGKGHDGLYQGLSTATKDTYDALHMQALPPR

SEQ ID NO: 139 - protein, 471 aa, Artificial Sequence
  anti-BCMA CAR
DIVMTQSPDSLAVSLGERATINCKSSQSVLYSSNNKNYLAWYQQKPGQPPKLLIYWASTRESGVPDRFSGSGSGTDFTLTISSLQAEDVAVYYCQQFAHTPFTFGGGTKVEIKRGSTSGSGKPGSGEGSTKGQVQLVQSGAEVKKPGSSVKVSCKASGGTFSSYAISWVRQAPGQGLEWMGGIIPIFGTANYAQKFQGRVTITADESTSTAYMELSSLRSEDTAVYYCARTPEYSSSIWHYYYGMDVWGQGTTVTVSSAAALDNEKSNGTIIHVKGKHLCPSPLFPGPSKPFWVLVVVGGVLACYSLLVTVAFIIFWVRSKRSRLLHSDYMNMTPRRPGPTRKHYQPYAPPRDFAAYRSRVKFSRSADAPAYQQGQNQLYNELNLGRREEYDVLDKRRGRDPEMGGKPRRKNPQEGLYNELQKDKMAEAYSEIGMKGERRRGKGHDGLYQGLSTATKDTYDALHMQALPPR

SEQ ID NO: 140 - protein, 462 aa, Artificial Sequence
  anti-BCMA CAR
QVQLVESGGGVVQPGRSLRLSCAASGFTFSSYGMHWVRQAPGKGLEWVAVISYDGSNKYYADSVKGRFTISRDNSKNTLYLQMNSLRAEDTAVYYCVKGPLQEPPYDYGMDVWGQGTTVTVSSGSTSGSGKPGSGEGSTKGEIVMTQSPATLSVSPGERATLSCRASQSVSSNLAWYQQKPGQAPRLLIYSASTRATGIPARFSGSGSGTEFTLTISSLQSEDFAVYYCQQHHVWPLTFGGGTKVEIKRAAALDNEKSNGTIIHVKGKHLCPSPLFPGPSKPFWVLVVVGGVLACYSLLVTVAFIIFWVRSKRSRLLHSDYMNMTPRRPGPTRKHYQPYAPPRDFAAYRSRVKFSRSADAPAYQQGQNQLYNELNLGRREEYDVLDKRRGRDPEMGGKPRRKNPQEGLYNELQKDKMAEAYSEIGMKGERRRGKGHDGLYQGLSTATKDTYDALHMQALPPR

SEQ ID NO: 141 - protein, 462 aa, Artificial Sequence
  anti-BCMA CAR
EIVMTQSPATLSVSPGERATLSCRASQSVSSNLAWYQQKPGQAPRLLIYSASTRATGIPARFSGSGSGTEFTLTISSLQSEDFAVYYCQQHHVWPLTFGGGTKVEIKRGSTSGSGKPGSGEGSTKGQVQLVESGGGVVQPGRSLRLSCAASGFTFSSYGMHWVRQAPGKGLEWVAVISYDGSNKYYADSVKGRFTISRDNSKNTLYLQMNSLRAEDTAVYYCVKGPLQEPPYDYGMDVWGQGTTVTVSSAAALDNEKSNGTIIHVKGKHLCPSPLFPGPSKPFWVLVVVGGVLACYSLLVTVAFIIFWVRSKRSRLLHSDYMNMTPRRPGPTRKHYQPYAPPRDFAAYRSRVKFSRSADAPAYQQGQNQLYNELNLGRREEYDVLDKRRGRDPEMGGKPRRKNPQEGLYNELQKDKMAEAYSEIGMKGERRRGKGHDGLYQGLSTATKDTYDALHMQALPPR

SEQ ID NO: 142 - protein, 466 aa, Artificial Sequence
  anti-BCMA CAR
QSALTQPASVSASPGQSIAISCTGTSSDVGWYQQHPGKAPKLMIYEDSKRPSGVSNRFSGSKSGNTASLTISGLQAEDEADYYCSSNTRSSTLVFGGGTKLTVLGSRGGGGSGGGGSGGGGSLEMAEVQLVQSGAEMKKPGASLKLSCKASGYTFIDYYVYWMRQAPGQGLESMGWINPNSGGTNYAQKFQGRVTMTRDTSISTAYMELSRLRSDDTAMYYCARSQRDGYMDYWGQGTLVTVSSAAAIEVMYPPPYLDNEKSNGTIIHVKGKHLCPSPLFPGPSKPFWVLVVVGGVLACYSLLVTVAFIIFWVRSKRSRLLHSDYMNMTPRRPGPTRKHYQPYAPPRDFAAYRSRVKFSRSADAPAYQQGQNQLYNELNLGRREEYDVLDKRRGRDPEMGGKPRRKNPQEGLYNELQKDKMAEAYSEIGMKGERRRGKGHDGLYQGLSTATKDTYDALHMQALPPR

SEQ ID NO: 143 - protein, 473 aa, Artificial Sequence
  anti-BCMA CAR
QSVLTQPPSVSGAPGQRVTISCTGSSSNIGAGFDVHWYQQLPGTAPKLLIYGNSNRPSGVPDRFSGSKSGTSASLAITGLQAEDEADYYCQSYDSSLSGYVFGTGTKVTVLGSRGGGGSGGGGSGGGGSLEMAQVQLVQSGAEVKKPGASVKVSCKASGYTFTDYYMHWVRQAPGQRLEWMGWINPNSGGTNYAQKFQDRITVTRDTSSNTGYMELTRLRSDDTAVYYCARSPYSGVLDKWGQGTLVTVSSAAAIEVMYPPPYLDNEKSNGTIIHVKGKHLCPSPLFPGPSKPFWVLVVVGGVLACYSLLVTVAFIIFWVRSKRSRLLHSDYMNMTPRRPGPTRKHYQPYAPPRDFAAYRSRVKFSRSADAPAYQQGQNQLYNELNLGRREEYDVLDKRRGRDPEMGGKPRRKNPQEGLYNELQKDKMAEAYSEIGMKGERRRGKGHDGLYQGLSTATKDTYDALHMQALPPR

SEQ ID NO: 144 - protein, 470 aa, Artificial Sequence
  anti-BCMA CAR
SYELTQPPSASGTPGQRVTMSCSGTSSNIGSHSVNWYQQLPGTAPKLLIYTNNQRPSGVPDRFSGSKSGTSASLAISGLQSEDEADYYCAAWDGSLNGLVFGGGTKLTVLGSRGGGGSGGGGSGGGGSLEMAEVQLVQSGAEVKKPGESLKISCKGSGYSFTSYWIGWVRQMPGKGLEWMGIIYPGDSDTRYSPSFQGHVTISADKSISTAYLQWSSLKASDTAMYYCARYSGSFDNWGQGTLVTVSSAAAIEVMYPPPYLDNEKSNGTIIHVKGKHLCPSPLFPGPSKPFWVLVVVGGVLACYSLLVTVAFIIFWVRSKRSRLLHSDYMNMTPRRPGPTRKHYQPYAPPRDFAAYRSRVKFSRSADAPAYQQGQNQLYNELNLGRREEYDVLDKRRGRDPEMGGKPRRKNPQEGLYNELQKDKMAEAYSEIGMKGERRRGKGHDGLYQGLSTATKDTYDALHMQALPPR

SEQ ID NO: 145 - protein, 476 aa, Artificial Sequence
  anti-BCMA CAR
LPVLTQPPSASGTPGQRVTISCSGRSSNIGSNSVNWYRQLPGAAPKLLIYSNNQRPPGVPVRFSGSKSGTSASLAISGLQSEDEATYYCATWDDNLNVHYVFGTGTKVTVLGSRGGGGSGGGGSGGGGSLEMAQVQLVQSGAEVKKPGSSVKVSCKASGGTFSSYAISWVRQAPGQGLEWMGRIIPILGIANYAQKFQGRVTITADKSTSTAYMELSSLRSEDTAVYYCARGGYYSHDMWSEDWGQGTLVTVSSAAAIEVMYPPPYLDNEKSNGTIIHVKGKHLCPSPLFPGPSKPFWVLVVVGGVLACYSLLVTVAFIIFWVRSKRSRLLHSDYMNMTPRRPGPTRKHYQPYAPPRDFAAYRSRVKFSRSADAPAYQQGQNQLYNELNLGRREEYDVLDKRRGRDPEMGGKPRRKNPQEGLYNELQKDKMAEAYSEIGMKGERRRGKGHDGLYQGLSTATKDTYDALHMQALPPR

SEQ ID NO: 146 - protein, 475 aa, Artificial Sequence
  anti-BCMA CAR
QAVLTQPPSASGTPGQRVTISCSGSSSNIGSNYVFWYQQLPGTAPKLLIYSNNQRPSGVPDRFSGSKSGTSASLAISGLRSEDEADYYCAAWDDSLSASYVFGTGTKVTVLGSRGGGGSGGGGSGGGGSLEMAQVQLVQSGAEVKKPGSSVKVSCKASGGTFSSYAISWVRQAPGQGLEWMGRIIPILGTANYAQKFQGRVTITADESTSTAYMELSSLRSEDTAVYYCARSGYGSYRWEDSWGQGTLVTVSSAAAIEVMYPPPYLDNEKSNGTIIHVKGKHLCPSPLFPGPSKPFWVLVVVGGVLACYSLLVTVAFIIFWVRSKRSRLLHSDYMNMTPRRPGPTRKHYQPYAPPRDFAAYRSRVKFSRSADAPAYQQGQNQLYNELNLGRREEYDVLDKRRGRDPEMGGKPRRKNPQEGLYNELQKDKMAEAYSEIGMKGERRRGKGHDGLYQGLSTATKDTYDALHMQALPPR

SEQ ID NO: 147 - protein, 482 aa, Artificial Sequence
  anti-BCMA CAR
LPVLTQPPSASGTPGQRVTISCSGRSSNIGSNSVNWYRQLPGAAPKLLIYSNNQRPPGVPVRFSGSKSGTSASLAISGLQSEDEATYYCATWDDNLNVHYVFGTGTKVTVLGSRGGGGSGGGGSGGGGSLEMAQVQLVQSGAEVKKPGSSVKVSCKASGGTFSSYAISWVRQAPGQGLEWMGRIIPILGIANYAQKFQGRVTITADKSTSTAYMELSSLRSEDTAVYYCARGGYYSHDMWSEDWGQGTLVTVSSAAAPTTTPAPRPPTPAPTIASQPLSLRPEACRPAAGGAVHTRGLDFACDIYIWAPLAGTCGVLLLSLVITLYCNKRGRKKLLYIFKQPFMRPVQTTQEEDGCSCRFPEEEEGGCELRVKFSRSAEPPAYQQGQNQLYNELNLGRREEYDVLDKRRGRDPEMGGKPRRKNPQEGLYNELQKDKMAEAYSEIGMKGERRRGKGHDGLYQGLSTATKDTYDALHMQALPPR

SEQ ID NO: 148 - protein, 476 aa, Artificial Sequence
  anti-BCMA CAR
SYELTQPPSASGTPGQRVTMSCSGTSSNIGSHSVNWYQQLPGTAPKLLIYTNNQRPSGVPDRFSGSKSGTSASLAISGLQSEDEADYYCAAWDGSLNGLVFGGGTKLTVLGSRGGGGSGGGGSGGGGSLEMAEVQLVQSGAEVKKPGESLKISCKGSGYSFTSYWIGWVRQMPGKGLEWMGIIYPGDSDTRYSPSFQGHVTISADKSISTAYLQWSSLKASDTAMYYCARYSGSFDNWGQGTLVTVSSAAAPTTTPAPRPPTPAPTIASQPLSLRPEACRPAAGGAVHTRGLDFACDIYIWAPLAGTCGVLLLSLVITLYCNKRGRKKLLYIFKQPFMRPVQTTQEEDGCSCRFPEEEEGGCELRVKFSRSAEPPAYQQGQNQLYNELNLGRREEYDVLDKRRGRDPEMGGKPRRKNPQEGLYNELQKDKMAEAYSEIGMKGERRRGKGHDGLYQGLSTATKDTYDALHMQALPPR

SEQ ID NO: 149 - protein, 481 aa, Artificial Sequence
  anti-BCMA CAR
QAVLTQPPSASGTPGQRVTISCSGSSSNIGSNYVFWYQQLPGTAPKLLIYSNNQRPSGVPDRFSGSKSGTSASLAISGLRSEDEADYYCAAWDDSLSASYVFGTGTKVTVLGSRGGGGSGGGGSGGGGSLEMAQVQLVQSGAEVKKPGSSVKVSCKASGGTFSSYAISWVRQAPGQGLEWMGRIIPILGTANYAQKFQGRVTITADESTSTAYMELSSLRSEDTAVYYCARSGYGSYRWEDSWGQGTLVTVSSAAAPTTTPAPRPPTPAPTIASQPLSLRPEACRPAAGGAVHTRGLDFACDIYIWAPLAGTCGVLLLSLVITLYCNKRGRKKLLYIFKQPFMRPVQTTQEEDGCSCRFPEEEEGGCELRVKFSRSAEPPAYQQGQNQLYNELNLGRREEYDVLDKRRGRDPEMGGKPRRKNPQEGLYNELQKDKMAEAYSEIGMKGERRRGKGHDGLYQGLSTATKDTYDALHMQALPPR

SEQ ID NO: 150 - protein, 479 aa, Artificial Sequence
  anti-BCMA CAR
QSVLTQPPSVSGAPGQRVTISCTGSSSNIGAGFDVHWYQQLPGTAPKLLIYGNSNRPSGVPDRFSGSKSGTSASLAITGLQAEDEADYYCQSYDSSLSGYVFGTGTKVTVLGSRGGGGSGGGGSGGGGSLEMAQVQLVQSGAEVKKPGASVKVSCKASGYTFTDYYMHWVRQAPGQRLEWMGWINPNSGGTNYAQKFQDRITVTRDTSSNTGYMELTRLRSDDTAVYYCARSPYSGVLDKWGQGTLVTVSSAAAPTTTPAPRPPTPAPTIASQPLSLRPEACRPAAGGAVHTRGLDFACDIYIWAPLAGTCGVLLLSLVITLYCNKRGRKKLLYIFKQPFMRPVQTTQEEDGCSCRFPEEEEGGCELRVKFSRSAEPPAYQQGQNQLYNELNLGRREEYDVLDKRRGRDPEMGGKPRRKNPQEGLYNELQKDKMAEAYSEIGMKGERRRGKGHDGLYQGLSTATKDTYDALHMQALPPR

SEQ ID NO: 151 - protein, 472 aa, Artificial Sequence
  anti-BCMA CAR
QSALTQPASVSASPGQSIAISCTGTSSDVGWYQQHPGKAPKLMIYEDSKRPSGVSNRFSGSKSGNTASLTISGLQAEDEADYYCSSNTRSSTLVFGGGTKLTVLGSRGGGGSGGGGSGGGGSLEMAEVQLVQSGAEMKKPGASLKLSCKASGYTFIDYYVYWMRQAPGQGLESMGWINPNSGGTNYAQKFQGRVTMTRDTSISTAYMELSRLRSDDTAMYYCARSQRDGYMDYWGQGTLVTVSSAAAPTTTPAPRPPTPAPTIASQPLSLRPEACRPAAGGAVHTRGLDFACDIYIWAPLAGTCGVLLLSLVITLYCNKRGRKKLLYIFKQPFMRPVQTTQEEDGCSCRFPEEEEGGCELRVKFSRSAEPPAYQQGQNQLYNELNLGRREEYDVLDKRRGRDPEMGGKPRRKNPQEGLYNELQKDKMAEAYSEIGMKGERRRGKGHDGLYQGLSTATKDTYDALHMQALPPR

SEQ ID NO: 152 - protein, 472 aa, Artificial Sequence
  anti-BCMA CAR
DIVLTQSPPSLAMSLGKRATISCRASESVTILGSHLIHWYQQKPGQPPTLLIQLASNVQTGVPARFSGSGSRTDFTLTIDPVEEDDVAVYYCLQSRTIPRTFGGGTKLEIKGSTSGSGKPGSGEGSTKGQIQLVQSGPELKKPGETVKISCKASGYTFTDYSINWVKRAPGKGLKWMGWINTETREPAYAYDFRGRFAFSLETSASTAYLQINNLKYEDTATYFCALDYSYAMDYWGQGTSVTVSSAAATTTPAPRPPTPAPTIASQPLSLRPEACRPAAGGAVHTRGLDFACDIYIWAPLAGTCGVLLLSLVITLYCKRGRKKLLYIFKQPFMRPVQTTQEEDGCSCRFPEEEEGGCELRVKFSRSADAPAYQQGQNQLYNELNLGRREEYDVLDKRRGRDPEMGGKPRRKNPQEGLYNELQKDKMAEAYSEIGMKGERRRGKGHDGLYQGLSTATKDTYDALHMQALPPR

SEQ ID NO: 153 - protein, 472 aa, Artificial Sequence
  anti-BCMA CAR
DIVLTQSPASLAVSLGERATINCRASESVSVIGAHLIHWYQQKPGQPPKLLIYLASNLETGVPARFSGSGSGTDFTLTISSLQAEDAAIYYCLQSRIFPRTFGQGTKLEIKGSTSGSGKPGSGEGSTKGQVQLVQSGSELKKPGASVKVSCKASGYTFTDYSINWVRQAPGQGLEWMGWINTETREPAYAYDFRGRFVFSLDTSVSTAYLQISSLKAEDTAVYYCARDYSYAMDYWGQGTLVTVSSAAATTTPAPRPPTPAPTIASQPLSLRPEACRPAAGGAVHTRGLDFACDIYIWAPLAGTCGVLLLSLVITLYCKRGRKKLLYIFKQPFMRPVQTTQEEDGCSCRFPEEEEGGCELRVKFSRSADAPAYQQGQNQLYNELNLGRREEYDVLDKRRGRDPEMGGKPRRKNPQEGLYNELQKDKMAEAYSEIGMKGERRRGKGHDGLYQGLSTATKDTYDALHMQALPPR

SEQ ID NO: 154 - protein, 466 aa, Artificial Sequence
  anti-BCMA CAR
DIVLTQSPASLAVSLGERATINCRASESVSVIGAHLIHWYQQKPGQPPKLLIYLASNLETGVPARFSGSGSGTDFTLTISSLQAEDAAIYYCLQSRIFPRTFGQGTKLEIKGSTSGSGKPGSGEGSTKGQVQLVQSGSELKKPGASVKVSCKASGYTFTDYSINWVRQAPGQGLEWMGWINTETREPAYAYDFRGRFVFSLDTSVSTAYLQISSLKAEDTAVYYCARDYSYAMDYWGQGTLVTVSSAAADTGLYICKVELMYPPPYYLGIGNGTQIYVIDPEPCPDSDFLLWILAAVSSGLFFYSFLLTAVSKRGRKKLLYIFKQPFMRPVQTTQEEDGCSCRFPEEEEGGCELRVKFSRSADAPAYQQGQNQLYNELNLGRREEYDVLDKRRGRDPEMGGKPRRKNPQEGLYNELQKDKMAEAYSEIGMKGERRRGKGHDGLYQGLSTATKDTYDALHMQALPPR

SEQ ID NO: 155 - protein, 464 aa, Artificial Sequence
  anti-BCMA CAR
DIVLTQSPASLAVSLGERATINCRASESVSVIGAHLIHWYQQKPGQPPKLLIYLASNLETGVPARFSGSGSGTDFTLTISSLQAEDAAIYYCLQSRIFPRTFGQGTKLEIKGSTSGSGKPGSGEGSTKGQVQLVQSGSELKKPGASVKVSCKASGYTFTDYSINWVRQAPGQGLEWMGWINTETREPAYAYDFRGRFVFSLDTSVSTAYLQISSLKAEDTAVYYCARDYSYAMDYWGQGTLVTVSSAAAQIKESLRAELRVTERRAEVPTAHPSPSPRPAGQFQTLVVGVVGGLLGSLVLLVWVLAVICSKRGRKKLLYIFKQPFMRPVQTTQEEDGCSCRFPEEEEGGCELRVKFSRSADAPAYQQGQNQLYNELNLGRREEYDVLDKRRGRDPEMGGKPRRKNPQEGLYNELQKDKMAEAYSEIGMKGERRRGKGHDGLYQGLSTATKDTYDALHMQALPPR

SEQ ID NO: 156 - protein, 653 aa, Artificial Sequence
  anti-BCMA CAR
EVQLVESGGGLVKPGGSLRLSCAASGFTFSDYYMSWIRQAPGKGLEWVSYISSSGSTIYYADSVKGRFTISRDNAKNSLYLQMNSLRAEDTAVYYCAKVDGDYTEDYWGQGTLVTVSSGGGGSGGGGSGGGGSQSALTQPASVSGSPGQSITISCTGSSSDVGKYNLVSWYQQPPGKAPKLIIYDVNKRPSGVSNRFSGSKSGNTATLTISGLQGDDEADYYCSSYGGSRSYVFGTGTKVTVLESKYGPPCPPCPAPPVAGPSVFLFPPKPKDTLMISRTPEVTCVVVDVSQEDPEVQFNWYVDGVEVHNAKTKPREEQFQSTYRVVSVLTVLHQDWLNGKEYKCKVSNKGLPSSIEKTISKAKGQPREPQVYTLPPSQEEMTKNQVSLTCLVKGFYPSDIAVEWESNGQPENNYKTTPPVLDSDGSFFLYSRLTVDKSRWQEGNVFSCSVMHEALHNHYTQKSLSLSLGKMFWVLVVVGGVLACYSLLVTVAFIIFWVKRGRKKLLYIFKQPFMRPVQTTQEEDGCSCRFPEEEEGGCELRVKFSRSADAPAYQQGQNQLYNELNLGRREEYDVLDKRRGRDPEMGGKPRRKNPQEGLYNELQKDKMAEAYSEIGMKGERRRGKGHDGLYQGLSTATKDTYDALHMQALPPR

SEQ ID NO: 157 - protein, 650 aa, Artificial Sequence
  anti-BCMA CAR
EVQLVQSGGGLVQPGRSLRLSCTASGFTFGDYAMSWFKQAPGKGLEWVGFIRSKAYGGTTEYAASVKGRFTISRDDSKSIAYLQMNSLKTEDTAVYYCAAWSAPTDYWGQGTLVTVSSGGGGSGGGGSGGGGSDIQMTQSPAFLSASVGDRVTVTCRASQGISNYLAWYQQKPGNAPRLLIYSASTLQSGVPSRFRGTGYGTEFSLTIDSLQPEDFATYYCQQSYTSRQTFGPGTRLDIKESKYGPPCPPCPAPPVAGPSVFLFPPKPKDTLMISRTPEVTCVVVDVSQEDPEVQFNWYVDGVEVHNAKTKPREEQFQSTYRVVSVLTVLHQDWLNGKEYKCKVSNKGLPSSIEKTISKAKGQPREPQVYTLPPSQEEMTKNQVSLTCLVKGFYPSDIAVEWESNGQPENNYKTTPPVLDSDGSFFLYSRLTVDKSRWQEGNVFSCSVMHEALHNHYTQKSLSLSLGKMFWVLVVVGGVLACYSLLVTVAFIIFWVKRGRKKLLYIFKQPFMRPVQTTQEEDGCSCRFPEEEEGGCELRVKFSRSADAPAYQQGQNQLYNELNLGRREEYDVLDKRRGRDPEMGGKPRRKNPQEGLYNELQKDKMAEAYSEIGMKGERRRGKGHDGLYQGLSTATKDTYDALHMQALPPR

SEQ ID NO: 158 - protein, 651 aa, Artificial Sequence
  anti-BCMA CAR
EVQLVESGGGLVKPGGSLRLSCAASGFTFSDYYMSWIRQAPGKGLEWVSYISSSGSTIYYADSVKGRFTISRDNAKNSLYLQMNSLRAEDTAVYYCAKVDGPPSFDIWGQGTMVTVSSGGGGSGGGGSGGGGSSYVLTQPPSVSVAPGQTARITCGANNIGSKSVHWYQQKPGQAPMLVVYDDDDRPSGIPERFSGSNSGNTATLTISGVEAGDEADYFCHLWDRSRDHYVFGTGTKLTVLESKYGPPCPPCPAPPVAGPSVFLFPPKPKDTLMISRTPEVTCVVVDVSQEDPEVQFNWYVDGVEVHNAKTKPREEQFQSTYRVVSVLTVLHQDWLNGKEYKCKVSNKGLPSSIEKTISKAKGQPREPQVYTLPPSQEEMTKNQVSLTCLVKGFYPSDIAVEWESNGQPENNYKTTPPVLDSDGSFFLYSRLTVDKSRWQEGNVFSCSVMHEALHNHYTQKSLSLSLGKMFWVLVVVGGVLACYSLLVTVAFIIFWVKRGRKKLLYIFKQPFMRPVQTTQEEDGCSCRFPEEEEGGCELRVKFSRSADAPAYQQGQNQLYNELNLGRREEYDVLDKRRGRDPEMGGKPRRKNPQEGLYNELQKDKMAEAYSEIGMKGERRRGKGHDGLYQGLSTATKDTYDALHMQALPPR

SEQ ID NO: 159 - protein, 658 aa, Artificial Sequence
  anti-BCMA CAR
SYELTQPPSASGTPGQRVTMSCSGTSSNIGSHSVNWYQQLPGTAPKLLIYTNNQRPSGVPDRFSGSKSGTSASLAISGLQSEDEADYYCAAWDGSLNGLVFGGGTKLTVLGSRGGGGSGGGGSGGGGSLEMAEVQLVQSGAEVKKPGESLKISCKGSGYSFTSYWIGWVRQMPGKGLEWMGIIYPGDSDTRYSPSFQGHVTISADKSISTAYLQWSSLKASDTAMYYCARYSGSFDNWGQGTLVTVSSESKYGPPCPPCPAPPVAGPSVFLFPPKPKDTLMISRTPEVTCVVVDVSQEDPEVQFNWYVDGVEVHNAKTKPREEQFQSTYRVVSVLTVLHQDWLNGKEYKCKVSNKGLPSSIEKTISKAKGQPREPQVYTLPPSQEEMTKNQVSLTCLVKGFYPSDIAVEWESNGQPENNYKTTPPVLDSDGSFFLYSRLTVDKSRWQEGNVFSCSVMHEALHNHYTQKSLSLSLGKMFWVLVVVGGVLACYSLLVTVAFIIFWVKRGRKKLLYIFKQPFMRPVQTTQEEDGCSCRFPEEEEGGCELRVKFSRSADAPAYQQGQNQLYNELNLGRREEYDVLDKRRGRDPEMGGKPRRKNPQEGLYNELQKDKMAEAYSEIGMKGERRRGKGHDGLYQGLSTATKDTYDALHMQALPPR

SEQ ID NO: 160 - protein, 654 aa, Artificial Sequence
  anti-BCMA CAR
QSALTQPASVSASPGQSIAISCTGTSSDVGWYQQHPGKAPKLMIYEDSKRPSGVSNRFSGSKSGNTASLTISGLQAEDEADYYCSSNTRSSTLVFGGGTKLTVLGSRGGGGSGGGGSGGGGSLEMAEVQLVQSGAEMKKPGASLKLSCKASGYTFIDYYVYWMRQAPGQGLESMGWINPNSGGTNYAQKFQGRVTMTRDTSISTAYMELSRLRSDDTAMYYCARSQRDGYMDYWGQGTLVTVSSESKYGPPCPPCPAPPVAGPSVFLFPPKPKDTLMISRTPEVTCVVVDVSQEDPEVQFNWYVDGVEVHNAKTKPREEQFQSTYRVVSVLTVLHQDWLNGKEYKCKVSNKGLPSSIEKTISKAKGQPREPQVYTLPPSQEEMTKNQVSLTCLVKGFYPSDIAVEWESNGQPENNYKTTPPVLDSDGSFFLYSRLTVDKSRWQEGNVFSCSVMHEALHNHYTQKSLSLSLGKMFWVLVVVGGVLACYSLLVTVAFIIFWVKRGRKKLLYIFKQPFMRPVQTTQEEDGCSCRFPEEEEGGCELRVKFSRSADAPAYQQGQNQLYNELNLGRREEYDVLDKRRGRDPEMGGKPRRKNPQEGLYNELQKDKMAEAYSEIGMKGERRRGKGHDGLYQGLSTATKDTYDALHMQALPPR

SEQ ID NO: 161 - protein, 653 aa, Artificial Sequence
  anti-BCMA CAR
QSALTQPASVSASPGQSIAISCTGTSSDVGWYQQHPGKAPKLMIYEDSKRPSGVSNRFSGSKSGNTASLTISGLQAEDEADYYCSSNTRSSTLVFGGGTKLTVLGSRGGGGSGGGGSGGGGSLEMAEVQLVQSGAEMKKPGASLKLSCKASGYTFIDYYVYWMRQAPGQGLESMGWINPNSGGTNYAQKFQGRVTMTRDTSISTAYMELSRLRSDDTAMYYCARSQRDGYMDYWGQGTLVTVSSESKYGPPCPPCPAPPVAGPSVFLFPPKPKDTLMISRTPEVTCVVVDVSQEDPEVQFNWYVDGVEVHNAKTKPREEQFQSTYRVVSVLTVLHQDWLNGKEYKCKVSNKGLPSSIEKTISKAKGQPREPQVYTLPPSQEEMTKNQVSLTCLVKGFYPSDIAVEWESNGQPENNYKTTPPVLDSDGSFFLYSRLTVDKSRWQEGNVFSCSVMHEALHNHYTQKSLSLSLGKMFWVLVVVGGVLACYSLLVTVAFIIFWVRSKRSRLLHSDYMNMTPRRPGPTRKHYQPYAPPRDFAAYRSRVKFSRSADAPAYQQGQNQLYNELNLGRREEYDVLDKRRGRDPEMGGKPRRKNPQEGLYNELQKDKMAEAYSEIGMKGERRRGKGHDGLYQGLSTATKDTYDALHMQALPPR

SEQ ID NO: 162 - protein, 462 aa, Artificial Sequence
  anti-BCMA CAR
EVQLVESGGGLVQPGGSLRLSCAVSGFALSNHGMSWVRRAPGKGLEWVSGIVYSGSTYYAASVKGRFTISRDNSRNTLYLQMNSLRPEDTAIYYCSAHGGESDVWGQGTTVTVSSASGGGGSGGRASGGGGSDIQLTQSPSSLSASVGDRVTITCRASQSISSYLNWYQQKPGKAPKLLIYAASSLQSGVPSRFSGSGSGTDFTLTISSLQPEDFATYYCQQSYSTPYTFGQGTKVEIKTTTPAPRPPTPAPTIASQPLSLRPEACRPAAGGAVHTRGLDFACDIYIWAPLAGTCGVLLLSLVITLYCKRGRKKLLYIFKQPFMRPVQTTQEEDGCSCRFPEEEEGGCELRVKFSRSADAPAYKQGQNQLYNELNLGRREEYDVLDKRRGRDPEMGGKPRRKNPQEGLYNELQKDKMAEAYSEIGMKGERRRGKGHDGLYQGLSTATKDTYDALHMQALPPR

SEQ ID NO: 163 - protein, 469 aa, Artificial Sequence
  anti-BCMA CAR
QVQLVESGGGLVQPGRSLRLSCAASGFTFSNYAMSWVRQAPGKGLGWVSGISRSGENTYYADSVKGRFTISRDNSKNTLYLQMNSLRDEDTAVYYCARSPAHYYGGMDVWGQGTTVTVSSASGGGGSGGRASGGGGSDIVLTQSPGTLSLSPGERATLSCRASQSISSSFLAWYQQKPGQAPRLLIYGASRRATGIPDRFSGSGSGTDFTLTISRLEPEDSAVYYCQQYHSSPSWTFGQGTKLEIKTTTPAPRPPTPAPTIASQPLSLRPEACRPAAGGAVHTRGLDFACDIYIWAPLAGTCGVLLLSLVITLYCKRGRKKLLYIFKQPFMRPVQTTQEEDGCSCRFPEEEEGGCELRVKFSRSADAPAYKQGQNQLYNELNLGRREEYDVLDKRRGRDPEMGGKPRRKNPQEGLYNELQKDKMAEAYSEIGMKGERRRGKGHDGLYQGLSTATKDTYDALHMQALPPR

SEQ ID NO: 164 - protein, 462 aa, Artificial Sequence
  anti-BCMA CAR
QVQLVESGGGLVQPGGSLRLSCAVSGFALSNHGMSWVRRAPGKGLEWVSGIVYSGSTYYAASVKGRFTISRDNSRNTLYLQMNSLRPEDTAIYYCSAHGGESDVWGQGTTVTVSSASGGGGSGGRASGGGGSDIRLTQSPSPLSASVGDRVTITCQASEDINKFLNWYHQTPGKAPKLLIYDASTLQTGVPSRFSGSGSGTDFTLTINSLQPEDIGTYYCQQYESLPLTFGGGTKVEIKTTTPAPRPPTPAPTIASQPLSLRPEACRPAAGGAVHTRGLDFACDIYIWAPLAGTCGVLLLSLVITLYCKRGRKKLLYIFKQPFMRPVQTTQEEDGCSCRFPEEEEGGCELRVKFSRSADAPAYKQGQNQLYNELNLGRREEYDVLDKRRGRDPEMGGKPRRKNPQEGLYNELQKDKMAEAYSEIGMKGERRRGKGHDGLYQGLSTATKDTYDALHMQALPPR

SEQ ID NO: 165 - protein, 464 aa, Artificial Sequence
  anti-BCMA CAR
EVQLVESGGGLVQPGGSLRLSCAVSGFALSNHGMSWVRRAPGKGLEWVSGIVYSGSTYYAASVKGRFTISRDNSRNTLYLQMNSLRPEDTAIYYCSAHGGESDVWGQGTTVTVSSASGGGGSGGRASGGGGSEIVLTQSPGTLSLSPGERATLSCRASQSIGSSSLAWYQQKPGQAPRLLMYGASSRASGIPDRFSGSGSGTDFTLTISRLEPEDFAVYYCQQYAGSPPFTFGQGTKVEIKTTTPAPRPPTPAPTIASQPLSLRPEACRPAAGGAVHTRGLDFACDIYIWAPLAGTCGVLLLSLVITLYCKRGRKKLLYIFKQPFMRPVQTTQEEDGCSCRFPEEEEGGCELRVKFSRSADAPAYKQGQNQLYNELNLGRREEYDVLDKRRGRDPEMGGKPRRKNPQEGLYNELQKDKMAEAYSEIGMKGERRRGKGHDGLYQGLSTATKDTYDALHMQALPPR

SEQ ID NO: 166 - protein, 467 aa, Artificial Sequence
  anti-BCMA CAR
QIQLVQSGPDLKKPGETVKLSCKASGYTFTNFGMNWVKQAPGKGFKWMAWINTYTGESYFADDFKGRFAFSVETSATTAYLQINNLKTEDTATYFCARGEIYYGYDGGFAYWGQGTLVTVSAGGGGSGGGGSGGGGSDVVMTQSHRFMSTSVGDRVSITCRASQDVNTAVSWYQQKPGQSPKLLIFSASYRYTGVPDRFTGSGSGADFTLTISSVQAEDLAVYYCQQHYSTPWTFGGGTKLDIKTTTPAPRPPTPAPTIASQPLSLRPEACRPAAGGAVHTRGLDFACDIYIWAPLAGTCGVLLLSLVITLYCKRGRKKLLYIFKQPFMRPVQTTQEEDGCSCRFPEEEEGGCELRVKFSRSADAPAYKQGQNQLYNELNLGRREEYDVLDKRRGRDPEMGGKPRRKNPQEGLYNELQKDKMAEAYSEIGMKGERRRGKGHDGLYQGLSTATKDTYDALHMQALPPR

SEQ ID NO: 167 - protein, 472 aa, Artificial Sequence
  anti-BCMA CAR
QIQLVQSGPELKKPGETVKISCKASGYTFTDYSINWVKRAPGKGLKWMGWINTETREPAYAYDFRGRFAFSLETSASTAYLQINNLKYEDTATYFCALDYSYAMDYWGQGTSVTVSSGGGGSGGGGSGGGGSQIQLVQSGPELKKPGETVKISCKASGYTFTDYSINWVKRAPGKGLKWMGWINTETREPAYAYDFRGRFAFSLETSASTAYLQINNLKYEDTATYFCALDYSYAMDYWGQGTSVTVSSTTTPAPRPPTPAPTIASQPLSLRPEACRPAAGGAVHTRGLDFACDIYIWAPLAGTCGVLLLSLVITLYCKRGRKKLLYIFKQPFMRPVQTTQEEDGCSCRFPEEEEGGCELRVKFSRSADAPAYKQGQNQLYNELNLGRREEYDVLDKRRGRDPEMGGKPRRKNPQEGLYNELQKDKMAEAYSEIGMKGERRRGKGHDGLYQGLSTATKDTYDALHMQALPPR

SEQ ID NO: 168 - protein, 466 aa, Artificial Sequence
  anti-BCMA CAR
QIQLVQSGPELKKPGETVKISCKASGYTFTDYSINWVKRAPGKGLKWMGWINTETREPAYAYDFRGRFAFSLETSASTAYLQINNLKYEDTATYFCALDYSYAMDYWGQGTSVTVSSGGGGSGGGGSGGGGSDIVLTQSPASLAMSLGKRATISCRASESVSVIGAHLIHWYQQKPGQPPKLLIYLASNLETGVPARFSGSGSGTDFTLTIDPVEEDDVAIYSCLQSRIFPRTFGGGTKLEIKTTTPAPRPPTPAPTIASQPLSLRPEACRPAAGGAVHTRGLDFACDIYIWAPLAGTCGVLLLSLVITLYCKRGRKKLLYIFKQPFMRPVQTTQEEDGCSCRFPEEEEGGCELRVKFSRSADAPAYKQGQNQLYNELNLGRREEYDVLDKRRGRDPEMGGKPRRKNPQEGLYNELQKDKMAEAYSEIGMKGERRRGKGHDGLYQGLSTATKDTYDALHMQALPPR

SEQ ID NO: 169 - protein, 466 aa, Artificial Sequence
  anti-BCMA CAR
QIQLVQSGPELKKPGETVKISCKASGYTFRHYSMNWVKQAPGKGLKWMGRINTESGVPIYADDFKGRFAFSVETSASTAYLVINNLKDEDTASYFCSNDYLYSLDFWGQGTALTVSSGGGGSGGGGSGGGGSDIVLTQSPPSLAMSLGKRATISCRASESVTILGSHLIYWYQQKPGQPPTLLIQLASNVQTGVPARFSGSGSRTDFTLTIDPVEEDDVAVYYCLQSRTIPRTFGGGTKLEIKTTTPAPRPPTPAPTIASQPLSLRPEACRPAAGGAVHTRGLDFACDIYIWAPLAGTCGVLLLSLVITLYCKRGRKKLLYIFKQPFMRPVQTTQEEDGCSCRFPEEEEGGCELRVKFSRSADAPAYKQGQNQLYNELNLGRREEYDVLDKRRGRDPEMGGKPRRKNPQEGLYNELQKDKMAEAYSEIGMKGERRRGKGHDGLYQGLSTATKDTYDALHMQALPPR

SEQ ID NO: 170 - protein, 466 aa, Artificial Sequence
  anti-BCMA CAR
QIQLVQSGPELKKPGETVKISCKASGYTFTHYSMNWVKQAPGKGLKWMGRINTETGEPLYADDFKGRFAFSLETSASTAYLVINNLKNEDTATFFCSNDYLYSCDYWGQGTTLTVSSGGGGSGGGGSGGGGSDIVLTQSPPSLAMSLGKRATISCRASESVTILGSHLIYWYQQKPGQPPTLLIQLASNVQTGVPARFSGSGSRTDFTLTIDPVEEDDVAVYYCLQSRTIPRTFGGGTKLEIKTTTPAPRPPTPAPTIASQPLSLRPEACRPAAGGAVHTRGLDFACDIYIWAPLAGTCGVLLLSLVITLYCKRGRKKLLYIFKQPFMRPVQTTQEEDGCSCRFPEEEEGGCELRVKFSRSADAPAYKQGQNQLYNELNLGRREEYDVLDKRRGRDPEMGGKPRRKNPQEGLYNELQKDKMAEAYSEIGMKGERRRGKGHDGLYQGLSTATKDTYDALHMQALPPR

SEQ ID NO: 171 - protein, 482 aa, Artificial Sequence
  anti-BCMA CAR
DIVLTQSPPSLAMSLGKRATISCRASESVTILGSHLIHWYQQKPGQPPTLLIQLASNVQTGVPARFSGSGSRTDFTLTIDPVEEDDVAVYYCLQSRTIPRTFGGGTKLEIKGSTSGSGKPGSGEGSTKGQIQLVQSGPELKKPGETVKISCKASGYTFTDYSINWVKRAPGKGLKWMGWINTETREPAYAYDFRGRFAFSLETSASTAYLQINNLKYEDTATYFCALDYSYAMDYWGQGTSVTVSSFVPVFLPAKPTTTPAPRPPTPAPTIASQPLSLRPEACRPAAGGAVHTRGLDFACDIYIWAPLAGTCGVLLLSLVITLYCNHRNRSKRSRLLHSDYMNMTPRRPGPTRKHYQPYAPPRDFAAYRSRVKFSRSADAPAYQQGQNQLYNELNLGRREEYDVLDKRRGRDPEMGGKPRRKNPQEGLYNELQKDKMAEAYSEIGMKGERRRGKGHDGLYQGLSTATKDTYDALHMQALPPR

SEQ ID NO: 172 - protein, 440 aa, Artificial Sequence
  anti-BCMA CAR
QVQLVQSGAEVKKPGASVKVSCKASGYSFPDYYINWVRQAPGQGLEWMGWIYFASGNSEYNQKFTGRVTMTRDTSINTAYMELSSLTSEDTAVYFCASLYDYDWYFDVWGQGTMVTVSSGGGGSGGGGSGGGGSDIVMTQTPLSLSVTPGQPASISCKSSQSLVHSNGNTYLHWYLQKPGQSPQLLIYKVSNRFSGVPDRFSGSGSGTDFTLKISRVEAEDVGIYYCSQSSIYPWTFGQGTKLEIKGLAVSTISSFFPPGYQIYIWAPLAGTCGVLLLSLVITLYCKRGRKKLLYIFKQPFMRPVQTTQEEDGCSCRFPEEEEGGCELRVKFSRSADAPAYQQGQNQLYNELNLGRREEYDVLDKRRGRDPEMGGKPRRKNPQEGLYNELQKDKMAEAYSEIGMKGERRRGKGHDGLYQGLSTATKDTYDALHMQALPPR

SEQ ID NO: 173 - protein, 469 aa, Artificial Sequence
  anti-BCMA CAR
QVQLVQSGAEVKKPGASVKVSCKASGYSFPDYYINWVRQAPGQGLEWMGWIYFASGNSEYNQKFTGRVTMTRDTSINTAYMELSSLTSEDTAVYFCASLYDYDWYFDVWGQGTMVTVSSGGGGSGGGGSGGGGSDIVMTQTPLSLSVTPGQPASISCKSSQSLVHSNGNTYLHWYLQKPGQSPQLLIYKVSNRFSGVPDRFSGSGSGTDFTLKISRVEAEDVGIYYCSQSSIYPWTFGQGTKLEIKTTTPAPRPPTPAPTIASQPLSLRPEACRPAAGGAVHTRGLDFACDIYIWAPLAGTCGVLLLSLVITLYCKRGRKKLLYIFKQPFMRPVQTTQEEDGCSCRFPEEEEGGCELRVKFSRSADAPAYQQGQNQLYNELNLGRREEYDVLDKRRGRDPEMGGKPRRKNPQEGLYNELQKDKMAEAYSEIGMKGERRRGKGHDGLYQGLSTATKDTYDALHMQALPPR

SEQ ID NO: 174 - protein, 655 aa, Artificial Sequence
  anti-BCMA CAR
QVQLVQSGAEVKKPGASVKVSCKASGYSFPDYYINWVRQAPGQGLEWMGWIYFASGNSEYNQKFTGRVTMTRDTSINTAYMELSSLTSEDTAVYFCASLYDYDWYFDVWGQGTMVTVSSGGGGSGGGGSGGGGSDIVMTQTPLSLSVTPGQPASISCKSSQSLVHSNGNTYLHWYLQKPGQSPQLLIYKVSNRFSGVPDRFSGSGSGTDFTLKISRVEAEDVGIYYCSQSSIYPWTFGQGTKLEIKEPKSPDKTHTCPPCPAPPVAGPSVFLFPPKPKDTLMIARTPEVTCVVVDVSHEDPEVKFNWYVDGVEVHNAKTKPREEQYNSTYRVVSVLTVLHQDWLNGKEYKCKVSNKALPAPIEKTISKAKGQPREPQVYTLPPSRDELTKNQVSLTCLVKGFYPSDIAVEWESNGQPENNYKTTPPVLDSDGSFFLYSKLTVDKSRWQQGNVFSCSVMHEALHNHYTQKSLSLSPGKIYIWAPLAGTCGVLLLSLVITLYCKRGRKKLLYIFKQPFMRPVQTTQEEDGCSCRFPEEEEGGCELRVKFSRSADAPAYQQGQNQLYNELNLGRREEYDVLDKRRGRDPEMGGKPRRKNPQEGLYNELQKDKMAEAYSEIGMKGERRRGKGHDGLYQGLSTATKDTYDALHMQALPPR

SEQ ID NO: 175 - protein, 440 aa, Artificial Sequence
  anti-BCMA CAR
QVQLVQSGAEVKKPGASVKVSCKASGYSFPDYYINWVRQAPGQGLEWMGWIYFASGNSEYNQKFTGRVTMTRDTSSSTAYMELSSLRSEDTAVYFCASLYDYDWYFDVWGQGTMVTVSSGGGGSGGGGSGGGGSDIVMTQTPLSLSVTPGEPASISCKSSQSLVHSNGNTYLHWYLQKPGQSPQLLIYKVSNRFSGVPDRFSGSGSGADFTLKISRVEAEDVGVYYCAETSHVPWTFGQGTKLEIKGLAVSTISSFFPPGYQIYIWAPLAGTCGVLLLSLVITLYCKRGRKKLLYIFKQPFMRPVQTTQEEDGCSCRFPEEEEGGCELRVKFSRSADAPAYQQGQNQLYNELNLGRREEYDVLDKRRGRDPEMGGKPRRKNPQEGLYNELQKDKMAEAYSEIGMKGERRRGKGHDGLYQGLSTATKDTYDALHMQALPPR

SEQ ID NO: 176 - protein, 469 aa, Artificial Sequence
  anti-BCMA CAR
QVQLVQSGAEVKKPGASVKVSCKASGYSFPDYYINWVRQAPGQGLEWMGWIYFASGNSEYNQKFTGRVTMTRDTSSSTAYMELSSLRSEDTAVYFCASLYDYDWYFDVWGQGTMVTVSSGGGGSGGGGSGGGGSDIVMTQTPLSLSVTPGEPASISCKSSQSLVHSNGNTYLHWYLQKPGQSPQLLIYKVSNRFSGVPDRFSGSGSGADFTLKISRVEAEDVGVYYCAETSHVPWTFGQGTKLEIKTTTPAPRPPTPAPTIASQPLSLRPEACRPAAGGAVHTRGLDFACDIYIWAPLAGTCGVLLLSLVITLYCKRGRKKLLYIFKQPFMRPVQTTQEEDGCSCRFPEEEEGGCELRVKFSRSADAPAYQQGQNQLYNELNLGRREEYDVLDKRRGRDPEMGGKPRRKNPQEGLYNELQKDKMAEAYSEIGMKGERRRGKGHDGLYQGLSTATKDTYDALHMQALPPR

SEQ ID NO: 177 - protein, 655 aa, Artificial Sequence
  anti-BCMA CAR
QVQLVQSGAEVKKPGASVKVSCKASGYSFPDYYINWVRQAPGQGLEWMGWIYFASGNSEYNQKFTGRVTMTRDTSSSTAYMELSSLRSEDTAVYFCASLYDYDWYFDVWGQGTMVTVSSGGGGSGGGGSGGGGSDIVMTQTPLSLSVTPGEPASISCKSSQSLVHSNGNTYLHWYLQKPGQSPQLLIYKVSNRFSGVPDRFSGSGSGADFTLKISRVEAEDVGVYYCAETSHVPWTFGQGTKLEIKEPKSPDKTHTCPPCPAPPVAGPSVFLFPPKPKDTLMIARTPEVTCVVVDVSHEDPEVKFNWYVDGVEVHNAKTKPREEQYNSTYRVVSVLTVLHQDWLNGKEYKCKVSNKALPAPIEKTISKAKGQPREPQVYTLPPSRDELTKNQVSLTCLVKGFYPSDIAVEWESNGQPENNYKTTPPVLDSDGSFFLYSKLTVDKSRWQQGNVFSCSVMHEALHNHYTQKSLSLSPGKIYIWAPLAGTCGVLLLSLVITLYCKRGRKKLLYIFKQPFMRPVQTTQEEDGCSCRFPEEEEGGCELRVKFSRSADAPAYQQGQNQLYNELNLGRREEYDVLDKRRGRDPEMGGKPRRKNPQEGLYNELQKDKMAEAYSEIGMKGERRRGKGHDGLYQGLSTATKDTYDALHMQALPPR

SEQ ID NO: 178 - protein, 28 aa, Artificial Sequence
  CD8a TM
IYIWAPLAGTCGVLLLSLVITLYCNHRN

SEQ ID NO: 179 - protein, 21 aa, Artificial Sequence
  CD8a TM
IYIWAPLAGTCGVLLLSLVIT

SEQ ID NO: 180 - protein, 4 aa, Artificial Sequence
  linking peptide
RAAA

SEQ ID NO: 181 - protein, 118 aa, Artificial Sequence
  Variable heavy (VH) Anti-BCMA
EVQLVESGGGLVKPGGSLRLSCAASGFTFSDYYMSWIRQAPGKGLEWVSYISSSGSTIYYADSVKGRFTISRDNAKNSLYLQMNSLRAEDTAVYYCAKVDGDYTEDYWGQGTLVTVSS

SEQ ID NO: 182 - protein, 110 aa, Artificial Sequence
  Variable light (VL) Anti-BCMA
QSALTQPASVSGSPGQSITISCTGSSSDVGKYNLVSWYQQPPGKAPKLIIYDVNKRPSGVSNRFSGSKSGNTATLTISGLQGDDEADYYCSSYGGSRSYVFGTGTKVTVL

SEQ ID NO: 183 - protein, 118 aa, Artificial Sequence
  Variable heavy (VH) Anti-BCMA
EVQLVQSGGGLVQPGRSLRLSCTASGFTFGDYAMSWFRQAPGKGLEWVGFIRSKAYGGTTEYAASVKGRFTISRDDSKSIAYLQMNSLKTEDTAVYYCAAWSAPTDYWGQGTLVTVSS

SEQ ID NO: 184 - protein, 107 aa, Artificial Sequence
  Variable light (VL) Anti-BCMA
DIQMTQSPAFLSASVGDRVTVTCRASQGISNYLAWYQQKPGNAPRLLIYSASTLQSGVPSRFRGTGYGTEFSLTIDSLQPEDFATYYCQQSYTSRQTFGPGTRLDIK

SEQ ID NO: 185 - protein, 118 aa, Artificial Sequence
  Variable heavy (VH) Anti-BCMA
EVQLVESGGGLVKPGGSLRLSCAASGFTFSDYYMSWIRQAPGKGLEWVSYISSSGSTIYYADSVKGRFTISRDNAKNSLYLQMNSLRAEDTAVYYCAKVDGPPSFDIWGQGTMVTVSS

SEQ ID NO: 186 - protein, 108 aa, Artificial Sequence
  Variable light (VL) Anti-BCMA
SYVLTQPPSVSVAPGQTARITCGANNIGSKSVHWYQQKPGQAPMLVVYDDDDRPSGIPERFSGSNSGNTATLTISGVEAGDEADYFCHLWDRSRDHYVFGTGTKLTVL

SEQ ID NO: 187 - protein, 122 aa, Artificial Sequence; identical to SEQ ID NO: 38
  Variable heavy (VH) Anti-BCMA

SEQ ID NO: 188 - protein, 111 aa, Artificial Sequence; identical to SEQ ID NO: 39
  Variable light (VL) Anti-BCMA

SEQ ID NO: 189 - protein, 17 aa, Artificial Sequence
  Linker
ASGGGGSGGRASGGGGS